European Patent Application EP 4 491 727 A1, published January 15, 2025. Title: LPA抑制剂及其用途. Applicant: 厦门甘宝利生物医药有限公司. The sequence listing filed with the application follows.

SEQUENCE LISTING (538 sequences)

SEQ ID NO: 1 - RNA, 21 nt, synthetic construct
  source 1..21: mol_type = other RNA
accacatggctttgctcaggt

SEQ ID NO: 2 - RNA, 21 nt, synthetic construct
  source 1..21: mol_type = other RNA
attatgttgatgtggtgtcat

SEQ ID NO: 3 - RNA, 21 nt, synthetic construct
  source 1..21: mol_type = other RNA
tcctattatgttgatgtggtg

SEQ ID NO: 4 - RNA, 21 nt, synthetic construct
  source 1..21: mol_type = other RNA
tttctgtggtcctattatgtt

SEQ ID NO: 5 - RNA, 21 nt, synthetic construct
  source 1..21: mol_type = other RNA
aataaggggctgccacaggat

SEQ ID NO: 6 - RNA, 21 nt, synthetic construct
  source 1..21: mol_type = other RNA
atagttggaggcgcgacggca

SEQ ID NO: 7 - RNA, 21 nt, synthetic construct
  source 1..21: mol_type = other RNA
aatagttggaggcgcgacggc

SEQ ID NO: 8 - RNA, 21 nt, synthetic construct
  source 1..21: mol_type = other RNA
taatagttggaggcgcgacgg

SEQ ID NO: 9 - RNA, 21 nt, synthetic construct
  source 1..21: mol_type = other RNA
taatgaagtatgtgccttgat

SEQ ID NO: 10 - RNA, 21 nt, synthetic construct
  source 1..21: mol_type = other RNA
acagtaatgaagtatgtgcct

SEQ ID NO: 11 - RNA, 21 nt, synthetic construct
  source 1..21: mol_type = other RNA
tcttcctgtgacagtaatgaa

SEQ ID NO: 12 - RNA, 21 nt, synthetic construct
  source 1..21: mol_type = other RNA
aggatctggatttcggcagta

SEQ ID NO: 13 - RNA, 21 nt, synthetic construct
  source 1..21: mol_type = other RNA
aacaccaaggggctgccacag

SEQ ID NO: 14 - RNA, 21 nt, synthetic construct
  source 1..21: mol_type = other RNA
ataacaccaaggggctgccac

SEQ ID NO: 15 - RNA, 21 nt, synthetic construct
  source 1..21: mol_type = other RNA
tgcatctgagcatcgtgtcag

SEQ ID NO: 16 - RNA, 21 nt, synthetic construct
  source 1..21: mol_type = other RNA
tctgcatctgagcatcgtgtc

SEQ ID NO: 17 - RNA, 21 nt, synthetic construct
  source 1..21: mol_type = other RNA
attctgcatctgagcatcgtg

SEQ ID NO: 18 - RNA, 21 nt, synthetic construct
  source 1..21: mol_type = other RNA
agtccattctgcatctgagca

SEQ ID NO: 19 - RNA, 21 nt, synthetic construct
  source 1..21: mol_type = other RNA
acattcggagggacgaaggca

SEQ ID NO: 20 - RNA, 21 nt, synthetic construct
  source 1..21: mol_type = other RNA
aacattcggagggacgaaggc

SEQ ID NO: 21 - RNA, 21 nt, synthetic construct
  source 1..21: mol_type = other RNA
aataacattcggagggacgaa

SEQ ID NO: 22 - RNA, 21 nt, synthetic construct
  source 1..21: mol_type = other RNA
aaagcctctaggcttggagcc

SEQ ID NO: 23 - RNA, 21 nt, synthetic construct
  source 1..21: mol_type = other RNA
aaaaagcctctaggcttggag

SEQ ID NO: 24 - RNA, 21 nt, synthetic construct
  source 1..21: mol_type = other RNA
aaaaaagcctctaggcttgga

SEQ ID NO: 25 - RNA, 21 nt, synthetic construct
  source 1..21: mol_type = other RNA
tcaaaaaaagcctctaggctt

SEQ ID NO: 26 - RNA, 21 nt, synthetic construct
  source 1..21: mol_type = other RNA
ttcaaaaaaagcctctaggct

SEQ ID NO: 27 - RNA, 21 nt, synthetic construct
  source 1..21: mol_type = other RNA
tgcttgttcaaaaaaagcctc

SEQ ID NO: 28 - RNA, 21 nt, synthetic construct
  source 1..21: mol_type = other RNA
agtgcttgttcaaaaaaagcc

SEQ ID NO: 29 - RNA, 21 nt, synthetic construct
  source 1..21: mol_type = other RNA
tttcctcagtcagtgcttgtt

SEQ ID NO: 30 - RNA, 21 nt, synthetic construct
  source 1..21: mol_type = other RNA
tagcagtcctgtaccccgggg

SEQ ID NO: 31 - RNA, 21 nt, synthetic construct
  source 1..21: mol_type = other RNA
agtagcagtcctgtaccccgg

SEQ ID NO: 32 - RNA, 21 nt, synthetic construct
  source 1..21: mol_type = other RNA
tagtagcagtcctgtaccccg

SEQ ID NO: 33 - RNA, 21 nt, synthetic construct
  source 1..21: mol_type = other RNA
aatggtagtagcagtcctgta

SEQ ID NO: 34 - RNA, 21 nt, synthetic construct
  source 1..21: mol_type = other RNA
ataatggtagtagcagtcctg

SEQ ID NO: 35 - RNA, 21 nt, synthetic construct
  source 1..21: mol_type = other RNA
tccataatggtagtagcagtc

SEQ ID NO: 36 - RNA, 21 nt, synthetic construct
  source 1..21: mol_type = other RNA
tgtccataatggtagtagcag

SEQ ID NO: 37 - RNA, 21 nt, synthetic construct
  source 1..21: mol_type = other RNA
actctgtccataatggtagta

SEQ ID NO: 38 - RNA, 21 nt, synthetic construct
  source 1..21: mol_type = other RNA
tctgtcaccaggcattgtgtc

SEQ ID NO: 39 - RNA, 21 nt, synthetic construct
  source 1..21: mol_type = other RNA
attctgtcaccaggcattgtg

SEQ ID NO: 40 - RNA, 21 nt, synthetic construct
  source 1..21: mol_type = other RNA
acttgattctgtcaccaggca

SEQ ID NO: 41 - RNA, 21 nt, synthetic construct
  source 1..21: mol_type = other RNA
agagttgcaaggacacttgat

SEQ ID NO: 42 - RNA, 21 nt, synthetic construct
  source 1..21: mol_type = other RNA
tggatctgggaccaccgtgag

SEQ ID NO: 43 - RNA, 21 nt, synthetic construct
  source 1..21: mol_type = other RNA
tcttcagaagaagcctctgtg

SEQ ID NO: 44 - RNA, 21 nt, synthetic construct
  source 1..21: mol_type = other RNA
tgcttcttcagaagaagcctc

SEQ ID NO: 45 - RNA, 21 nt, synthetic construct
  source 1..21: mol_type = other RNA
agcaatcctggaccccggggc

SEQ ID NO: 46 - RNA, 21 nt, synthetic construct
  source 1..21: mol_type = other RNA
tagcaatcctggaccccgggg

SEQ ID NO: 47 - RNA, 21 nt, synthetic construct
  source 1..21: mol_type = other RNA
tgttgtcctctgatgccagtg

SEQ ID NO: 48 - RNA, 21 nt, synthetic construct
  source 1..21: mol_type = other RNA
tctgttgtcctctgatgccag

SEQ ID NO: 49 - RNA, 21 nt, synthetic construct
  source 1..21: mol_type = other RNA
ttctgttgtcctctgatgcca

SEQ ID NO: 50 - RNA, 21 nt, synthetic construct
  source 1..21: mol_type = other RNA
attctgttgtcctctgatgcc

SEQ ID NO: 51 - RNA, 21 nt, synthetic construct
  source 1..21: mol_type = other RNA
aatattctgttgtcctctgat

SEQ ID NO: 52 - RNA, 21 nt, synthetic construct
  source 1..21: mol_type = other RNA
ataatattctgttgtcctctg

SEQ ID NO: 53 - RNA, 21 nt, synthetic construct
  source 1..21: mol_type = other RNA
tggataatattctgttgtcct

SEQ ID NO: 54 - RNA, 21 nt, synthetic construct
  source 1..21: mol_type = other RNA
tttggataatattctgttgtc

SEQ ID NO: 55 - RNA, 21 nt, synthetic construct
  source 1..21: mol_type = other RNA
aaggactaatctcagcatctg

SEQ ID NO: 56 - RNA, 21 nt, synthetic construct
  source 1..21: mol_type = other RNA
aacaccaaggactaatctcag

SEQ ID NO: 57 - RNA, 21 nt, synthetic construct
  source 1..21: mol_type = other RNA
ataacaccaaggactaatctc

SEQ ID NO: 58 - RNA, 21 nt, synthetic construct
  source 1..21: mol_type = other RNA
atggtataacaccaaggacta

SEQ ID NO: 59 - RNA, 21 nt, synthetic construct
  source 1..21: mol_type = other RNA
aaacagccgtggacgtcgcaa

SEQ ID NO: 60 - RNA, 21 nt, synthetic construct
  source 1..21: mol_type = other RNA
agaaacagccgtggacgtcgc

SEQ ID NO: 61 - RNA, 21 nt, synthetic construct
  source 1..21: mol_type = other RNA
tcagaaacagccgtggacgtc

SEQ ID NO: 62 - RNA, 21 nt, synthetic construct
  source 1..21: mol_type = other RNA
ttcagaaacagccgtggacgt

SEQ ID NO: 63 - RNA, 21 nt, synthetic construct
  source 1..21: mol_type = other RNA
tgttcagaaacagccgtggac

SEQ ID NO: 64 - RNA, 21 nt, synthetic construct
  source 1..21: mol_type = other RNA
ttgttcagaaacagccgtgga

SEQ ID NO: 65 - RNA, 21 nt, synthetic construct
  source 1..21: mol_type = other RNA
tgcttgttcagaaacagccgt

SEQ ID NO: 66 - RNA, 21 nt, synthetic construct
  source 1..21: mol_type = other RNA
tagcagtcctggactgtgggg

SEQ ID NO: 67 - RNA, 21 nt, synthetic construct
  source 1..21: mol_type = other RNA
tgtggttctctgatgccagtg

SEQ ID NO: 68 - RNA, 21 nt, synthetic construct
  source 1..21: mol_type = other RNA
attctgtggttctctgatgcc

SEQ ID NO: 69 - RNA, 21 nt, synthetic construct
  source 1..21: mol_type = other RNA
agtattctgtggttctctgat

SEQ ID NO: 70 - RNA, 21 nt, synthetic construct
  source 1..21: mol_type = other RNA
tccatcactggacattgcgtc

SEQ ID NO: 71 - RNA, 21 nt, synthetic construct
  source 1..21: mol_type = other RNA
ttccatcactggacattgcgt

SEQ ID NO: 72 - RNA, 21 nt, synthetic construct
  source 1..21: mol_type = other RNA
attccatcactggacattgcg

SEQ ID NO: 73 - RNA, 21 nt, synthetic construct
  source 1..21: mol_type = other RNA
agagttgattccatcactgga

SEQ ID NO: 74 - RNA, 21 nt, synthetic construct
  source 1..21: mol_type = other RNA
ttgtgaggagagttgattcca

SEQ ID NO: 75 - RNA, 21 nt, synthetic construct
  source 1..21: mol_type = other RNA
aaggaagctctgtgcttggaa

SEQ ID NO: 76 - RNA, 21 nt, synthetic construct
  source 1..21: mol_type = other RNA
tcagaaggaagctctgtgctt

SEQ ID NO: 77 - RNA, 21 nt, synthetic construct
  source 1..21: mol_type = other RNA
ttcagaaggaagctctgtgct

SEQ ID NO: 78 - RNA, 21 nt, synthetic construct
  source 1..21: mol_type = other RNA
tcttcagaaggaagctctgtg

SEQ ID NO: 79 - RNA, 21 nt, synthetic construct
  source 1..21: mol_type = other RNA
tgcttcttcagaaggaagctc

SEQ ID NO: 80 - RNA, 21 nt, synthetic construct
  source 1..21: mol_type = other RNA
tttcagttggtgcttcttcag

SEQ ID NO: 81 - RNA, 21 nt, synthetic construct
  source 1..21: mol_type = other RNA
tgttttcagttggtgcttctt

SEQ ID NO: 82 - RNA, 21 nt, synthetic construct
  source 1..21: mol_type = other RNA
tgctgttttcagttggtgctt

SEQ ID NO: 83 - RNA, 21 nt, synthetic construct
  source 1..21: mol_type = other RNA
tagcagtcctggaccccagtg

SEQ ID NO: 84 - RNA, 21 nt, synthetic construct
  source 1..21: mol_type = other RNA
atcacctcggtagcagtcctg

SEQ ID NO: 85 - RNA, 21 nt, synthetic construct
  source 1..21: mol_type = other RNA
tccatcacctcggtagcagtc

SEQ ID NO: 86 - RNA, 21 nt, synthetic construct
  source 1..21: mol_type = other RNA
tgtccatcacctcggtagcag

SEQ ID NO: 87 - RNA, 21 nt, synthetic construct
  source 1..21: mol_type = other RNA
actctgtccatcacctcggta

SEQ ID NO: 88 - RNA, 21 nt, synthetic construct
  source 1..21: mol_type = other RNA
aactctgtccatcacctcggt

SEQ ID NO: 89 - RNA, 21 nt, synthetic construct
  source 1..21: mol_type = other RNA
taactctgtccatcacctcgg

SEQ ID NO: 90 - RNA, 21 nt, synthetic construct
  source 1..21: mol_type = other RNA
atagtggtggagagtgtgcct

SEQ ID NO: 91 - RNA, 21 nt, synthetic construct
  source 1..21: mol_type = other RNA
aatgggatcctccgatgccaa

SEQ ID NO: 92 - RNA, 21 nt, synthetic construct
  source 1..21: mol_type = other RNA
taatgggatcctccgatgcca

SEQ ID NO: 93 - RNA, 21 nt, synthetic construct
  source 1..21: mol_type = other RNA
ataatgggatcctccgatgcc

SEQ ID NO: 94 - RNA, 21 nt, synthetic construct
  source 1..21: mol_type = other RNA
agtataatgggatcctccgat

SEQ ID NO: 95 - RNA, 21 nt, synthetic construct
  source 1..21: mol_type = other RNA
tagtataatgggatcctccga

SEQ ID NO: 96 - RNA, 21 nt, synthetic construct
  source 1..21: mol_type = other RNA
atagtataatgggatcctccg

SEQ ID NO: 97 - RNA, 21 nt, synthetic construct
  source 1..21: mol_type = other RNA
tggatagtataatgggatcct

SEQ ID NO: 98 - RNA, 21 nt, synthetic construct
  source 1..21: mol_type = other RNA
atttggatagtataatgggat

SEQ ID NO: 99 - RNA, 21 nt, synthetic construct
  source 1..21: mol_type = other RNA
ttgtgaggacactcgattctg

SEQ ID NO: 100 - RNA, 21 nt, synthetic construct
  source 1..21: mol_type = other RNA
tgtgcttggaaccggggccac

SEQ ID NO: 101 - RNA, 21 nt, synthetic construct
  source 1..21: mol_type = other RNA
ttttctcaggtggtgcttgtt

SEQ ID NO: 102 - RNA, 21 nt, synthetic construct
  source 1..21: mol_type = other RNA
atatgcctcgataactccgtc

SEQ ID NO: 103 - RNA, 21 nt, synthetic construct
  source 1..21: mol_type = other RNA
agttctcggtcaggccagcat

SEQ ID NO: 104 - RNA, 21 nt, synthetic construct
  source 1..21: mol_type = other RNA
tagttctcggtcaggccagca

SEQ ID NO: 105 - RNA, 21 nt, synthetic construct
  source 1..21: mol_type = other RNA
agtagttctcggtcaggccag

SEQ ID NO: 106 - RNA, 21 nt, synthetic construct
  source 1..21: mol_type = other RNA
tgcagtagttctcggtcaggc

SEQ ID NO: 107 - RNA, 21 nt, synthetic construct
  source 1..21: mol_type = other RNA
attcctgcagtagttctcggt

SEQ ID NO: 108 - RNA, 21 nt, synthetic construct
  source 1..21: mol_type = other RNA
tctaggacacctgattctgtt

SEQ ID NO: 109 - RNA, 21 nt, synthetic construct
  source 1..21: mol_type = other RNA
tctctaggacacctgattctg

SEQ ID NO: 110 - RNA, 21 nt, synthetic construct
  source 1..21: mol_type = other RNA
tcagaaggaggccctaggctt

SEQ ID NO: 111 - RNA, 21 nt, synthetic construct
  source 1..21: mol_type = other RNA
ttcagaaggaggccctaggct

SEQ ID NO: 112 - RNA, 21 nt, synthetic construct
  source 1..21: mol_type = other RNA
tcttgttcagaaggaggccct

SEQ ID NO: 113 - RNA, 21 nt, synthetic construct
  source 1..21: mol_type = other RNA
agtcttgttcagaaggaggcc

SEQ ID NO: 114 - RNA, 21 nt, synthetic construct
  source 1..21: mol_type = other RNA
tacagtcttgttcagaaggag

SEQ ID NO: 115 - RNA, 21 nt, synthetic construct
  source 1..21: mol_type = other RNA
atacagtcttgttcagaagga

SEQ ID NO: 116 - RNA, 21 nt, synthetic construct
  source 1..21: mol_type = other RNA
aacatacagtcttgttcagaa

SEQ ID NO: 117 - RNA, 21 nt, synthetic construct
  source 1..21: mol_type = other RNA
tttgtccctggaatgaacgtg

SEQ ID NO: 118 - RNA, 21 nt, synthetic construct
  source 1..21: mol_type = other RNA
atttgtccctggaatgaacgt

SEQ ID NO: 119 - RNA, 21 nt, synthetic construct
  source 1..21: mol_type = other RNA
tttatttgtccctggaatgaa

SEQ ID NO: 120 - RNA, 21 nt, synthetic construct
  source 1..21: mol_type = other RNA
atgtcaccatcagggttacgg

SEQ ID NO: 121 - RNA, 21 nt, synthetic construct
  source 1..21: mol_type = other RNA
attgatgtcaccatcagggtt

SEQ ID NO: 122 - RNA, 21 nt, synthetic construct
  source 1..21: mol_type = other RNA
attcattgtgtagcaccaggg

SEQ ID NO: 123 - RNA, 21 nt, synthetic construct
  source 1..21: mol_type = other RNA
tggattcattgtgtagcacca

SEQ ID NO: 124 - RNA, 21 nt, synthetic construct
  source 1..21: mol_type = other RNA
tcttggattcattgtgtagca

SEQ ID NO: 125 - RNA, 21 nt, synthetic construct
  source 1..21: mol_type = other RNA
ttttcttggattcattgtgta

SEQ ID NO: 126 - RNA, 21 nt, synthetic construct
  source 1..21: mol_type = other RNA
aaaaagttttcttggattcat

SEQ ID NO: 127 - RNA, 21 nt, synthetic construct
  source 1..21: mol_type = other RNA
agtcaaaaagttttcttggat

SEQ ID NO: 128 - RNA, 21 nt, synthetic construct
  source 1..21: mol_type = other RNA
tagtcaaaaagttttcttgga

SEQ ID NO: 129 - RNA, 21 nt, synthetic construct
  source 1..21: mol_type = other RNA
tatcacagtagtcaaaaagtt

SEQ ID NO: 130 - RNA, 21 nt, synthetic construct
  source 1..21: mol_type = other RNA
acagagagggatatcacagta

SEQ ID NO: 131 - RNA, 21 nt, synthetic construct
  source 1..21: mol_type = other RNA
aaatgaagaggatgcacagag

SEQ ID NO: 132 - RNA, 21 nt, synthetic construct
  source 1..21: mol_type = other RNA
aatgcttccaggacatttctt

SEQ ID NO: 133 - RNA, 21 nt, synthetic construct
  source 1..21: mol_type = other RNA
ttcaagcagtgagcagcagtc

SEQ ID NO: 134 - RNA, 21 nt, synthetic construct
  source 1..21: mol_type = other RNA
tcttcaagcagtgagcagcag

SEQ ID NO: 135 - RNA, 21 nt, synthetic construct
  source 1..21: mol_type = other RNA
ttcttcaagcagtgagcagca

SEQ ID NO: 136 - RNA, 21 nt, synthetic construct
  source 1..21: mol_type = other RNA
acttcttcaagcagtgagcag

SEQ ID NO: 137 - RNA, 21 nt, synthetic construct
  source 1..21: mol_type = other RNA
aggacttcttcaagcagtgag

SEQ ID NO: 138 - RNA, 21 nt, synthetic construct
  source 1..21: mol_type = other RNA
aacatgagattcgaggttcac

SEQ ID NO: 139 - RNA, 21 nt, synthetic construct
  source 1..21: mol_type = other RNA
ttcctgaacatgagattcgag

SEQ ID NO: 140 - RNA, 21 nt, synthetic construct
  source 1..21: mol_type = other RNA
tttcctgaacatgagattcga

SEQ ID NO: 141 - RNA, 21 nt, synthetic construct
  source 1..21: mol_type = other RNA
tctatttcctgaacatgagat

SEQ ID NO: 142 - RNA, 21 nt, synthetic construct
  source 1..21: mol_type = other RNA
tgcttgtgtgggctccaagaa

SEQ ID NO: 143 - RNA, 21 nt, synthetic construct
  source 1..21: mol_type = other RNA
atctgcttgtgtgggctccaa

SEQ ID NO: 144 - RNA, 21 nt, synthetic construct
  source 1..21: mol_type = other RNA
tatctgcttgtgtgggctcca

SEQ ID NO: 145 - RNA, 21 nt, synthetic construct
  source 1..21: mol_type = other RNA
aatatctgcttgtgtgggctc

SEQ ID NO: 146 - RNA, 21 nt, synthetic construct
  source 1..21: mol_type = other RNA
aaggcaatatctgcttgtgtg

SEQ ID NO: 147 - RNA, 21 nt, synthetic construct
  source 1..21: mol_type = other RNA
ttagcaaggcaatatctgctt

SEQ ID NO: 148 - RNA, 21 nt, synthetic construct
  source 1..21: mol_type = other RNA
tagtctggggatggcagacaa

SEQ ID NO: 149 - RNA, 21 nt, synthetic construct
  source 1..21: mol_type = other RNA
tgtagtctggggatggcagac

SEQ ID NO: 150 - RNA, 21 nt, synthetic construct
  source 1..21: mol_type = other RNA
accatgtagtctggggatggc

SEQ ID NO: 151 - RNA, 21 nt, synthetic construct
  source 1..21: mol_type = other RNA
ttcagtcctggcggtgaccat

SEQ ID NO: 152 - RNA, 21 nt, synthetic construct
  source 1..21: mol_type = other RNA
attcagtcctggcggtgacca

SEQ ID NO: 153 - RNA, 21 nt, synthetic construct
  source 1..21: mol_type = other RNA
acattcagtcctggcggtgac

SEQ ID NO: 154 - RNA, 21 nt, synthetic construct
  source 1..21: mol_type = other RNA
taacattcagtcctggcggtg

SEQ ID NO: 155 - RNA, 21 nt, synthetic construct
  source 1..21: mol_type = other RNA
tgtaacattcagtcctggcgg

SEQ ID NO: 156 - RNA, 21 nt, synthetic construct
  source 1..21: mol_type = other RNA
atgtaacattcagtcctggcg

SEQ ID NO: 157 - RNA, 21 nt, synthetic construct
  source 1..21: mol_type = other RNA
taacaaggagctgggcttcct

SEQ ID NO: 158 - RNA, 21 nt, synthetic construct
  source 1..21: mol_type = other RNA
tcaataacaaggagctgggct

SEQ ID NO: 159 - RNA, 21 nt, synthetic construct
  source 1..21: mol_type = other RNA
tctcaataacaaggagctggg

SEQ ID NO: 160 - RNA, 21 nt, synthetic construct
  source 1..21: mol_type = other RNA
attctcaataacaaggagctg

SEQ ID NO: 161 - RNA, 21 nt, synthetic construct
  source 1..21: mol_type = other RNA
ttcattctcaataacaaggag

SEQ ID NO: 162 - RNA, 21 nt, synthetic construct
  source 1..21: mol_type = other RNA
acacttcattctcaataacaa

SEQ ID NO: 163 - RNA, 21 nt, synthetic construct
  source 1..21: mol_type = other RNA
tatagtgattgcacacttcat

SEQ ID NO: 164 - RNA, 21 nt, synthetic construct
  source 1..21: mol_type = other RNA
acttatagtgattgcacactt

SEQ ID NO: 165 - RNA, 21 nt, synthetic construct
  source 1..21: mol_type = other RNA
atacttatagtgattgcacac

SEQ ID NO: 166 - RNA, 21 nt, synthetic construct
  source 1..21: mol_type = other RNA
atatacttatagtgattgcac

SEQ ID NO: 167 - RNA, 21 nt, synthetic construct
  source 1..21: mol_type = other RNA
aatatacttatagtgattgca

SEQ ID NO: 168 - RNA, 21 nt, synthetic construct
  source 1..21: mol_type = other RNA
agcacaaatatacttatagtg

SEQ ID NO: 169 - RNA, 21 nt, synthetic construct
  source 1..21: mol_type = other RNA
atgctcagcacaaatatactt

SEQ ID NO: 170 - RNA, 21 nt, synthetic construct
  source 1..21: mol_type = other RNA
tgatgcttcactctgtctccc

SEQ ID NO: 171 - RNA, 21 nt, synthetic construct
  source 1..21: mol_type = other RNA
aggttgatgcttcactctgtc

SEQ ID NO: 172 - RNA, 21 nt, synthetic construct
  source 1..21: mol_type = other RNA
aagtaggttgatgcttcactc

SEQ ID NO: 173 - RNA, 21 nt, synthetic construct
  source 1..21: mol_type = other RNA
tcagcttctaagtaggttgat

SEQ ID NO: 174 - RNA, 21 nt, synthetic construct
  source 1..21: mol_type = other RNA
ttacccacgtttcagcttcta

SEQ ID NO: 175 - RNA, 21 nt, synthetic construct
  source 1..21: mol_type = other RNA
tccttacccacgtttcagctt

SEQ ID NO: 176 - RNA, 21 nt, synthetic construct
  source 1..21: mol_type = other RNA
atccttacccacgtttcagct

SEQ ID NO: 177 - RNA, 21 nt, synthetic construct
  source 1..21: mol_type = other RNA
aaatccttacccacgtttcag

SEQ ID NO: 178 - RNA, 21 nt, synthetic construct
  source 1..21: mol_type = other RNA
attgctgtctattatttccag

SEQ ID NO: 179 - RNA, 21 nt, synthetic construct
  source 1..21: mol_type = other RNA
tcttcgtttgattgctgtcta

SEQ ID NO: 180 - RNA, 21 nt, synthetic construct
  source 1..21: mol_type = other RNA
atgccaaggtttggcatagct

SEQ ID NO: 181 - RNA, 21 nt, synthetic construct
  source 1..21: mol_type = other RNA
aaaaatgccaaggtttggcat

SEQ ID NO: 182 - RNA, 21 nt, synthetic construct
  source 1..21: mol_type = other RNA
aataccaaaaatgccaaggtt

SEQ ID NO: 183 - RNA, 21 nt, synthetic construct
  source 1..21: mol_type = other RNA
aaataccaaaaatgccaaggt

SEQ ID NO: 184 - RNA, 21 nt, synthetic construct
  source 1..21: mol_type = other RNA
acaaaaataccaaaaatgcca

SEQ ID NO: 185 - RNA, 21 nt, synthetic construct
  source 1..21: mol_type = other RNA
agcttatacacaaaaatacca

SEQ ID NO: 186 - RNA, 21 nt, synthetic construct
  source 1..21: mol_type = other RNA
accttaaaagcttatacacaa

SEQ ID NO: 187 - RNA, 21 nt, synthetic construct
  source 1..21: mol_type = other RNA
agaccttaaaagcttatacac

SEQ ID NO: 188 - RNA, 21 nt, synthetic construct
  source 1..21: mol_type = other RNA
tcagtcagaccttaaaagctt

SEQ ID NO: 189 - RNA, 21 nt, synthetic construct
  source 1..21: mol_type = other RNA
agaatttgtcagtcagacctt

SEQ ID NO: 190 - RNA, 21 nt, synthetic construct
  source 1..21: mol_type = other RNA
tacagaatttgtcagtcagac

SEQ ID NO: 191 - RNA, 21 nt, synthetic construct
  source 1..21: mol_type = other RNA
aatacagaatttgtcagtcag

SEQ ID NO: 192 - RNA, 21 nt, synthetic construct
  source 1..21: mol_type = other RNA
ttaatacagaatttgtcagtc

SEQ ID NO: 193 - RNA, 21 nt, synthetic construct
  source 1..21: mol_type = other RNA
agctatgacaccttaatacag

SEQ ID NO: 194 - RNA, 21 nt, synthetic construct
  source 1..21: mol_type = other RNA
aatcaaaataagtgcagagtt

SEQ ID NO: 195 - RNA, 21 nt, synthetic construct
  source 1..21: mol_type = other RNA
  misc_feature 21: note = n is a,g,c or u
ctgagcaaagccatgtggtcn

SEQ ID NO: 196 - RNA, 21 nt, synthetic construct
  source 1..21: mol_type = other RNA
  misc_feature 21: note = n is a,g,c or u
gacaccacatcaacataatan

SEQ ID NO: 197 - RNA, 21 nt, synthetic construct
  source 1..21: mol_type = other RNA
  misc_feature 21: note = n is a,g,c or u
ccacatcaacataataggacn

SEQ ID NO: 198 - RNA, 21 nt, synthetic construct
  source 1..21: mol_type = other RNA
  misc_feature 21: note = n is a,g,c or u
cataataggaccacagaaaan

SEQ ID NO: 199 - RNA, 21 nt, synthetic construct
  source 1..21: mol_type = other RNA
  misc_feature 21: note = n is a,g,c or u
cctgtggcagccccttattgn

SEQ ID NO: 200 - RNA, 21 nt, synthetic construct
  source 1..21: mol_type = other RNA
  misc_feature 21: note = n is a,g,c or u
ccgtcgcgcctccaactattn

SEQ ID NO: 201 - RNA, 21 nt, synthetic construct
  source 1..21: mol_type = other RNA
  misc_feature 21: note = n is a,g,c or u
cgtcgcgcctccaactattan

SEQ ID NO: 202 - RNA, 21 nt, synthetic construct
  source 1..21: mol_type = other RNA
  misc_feature 21: note = n is a,g,c or u
gtcgcgcctccaactattacn

SEQ ID NO: 203 - RNA, 21 nt, synthetic construct
  source 1..21: mol_type = other RNA
  misc_feature 21: note = n is a,g,c or u
caaggcacatacttcattacn

SEQ ID NO: 204 - RNA, 21 nt, synthetic construct
  source 1..21: mol_type = other RNA
  misc_feature 21: note = n is a,g,c or u
gcacatacttcattactgtcn

SEQ ID NO: 205 - RNA, 21 nt, synthetic construct
  source 1..21: mol_type = other RNA
  misc_feature 21: note = n is a,g,c or u
cattactgtcacaggaagaan

SEQ ID NO: 206 - RNA, 21 nt, synthetic construct
  source 1..21: mol_type = other RNA
  misc_feature 21: note = n is a,g,c or u
ctgccgaaatccagatcctgn

SEQ ID NO: 207 - RNA, 21 nt, synthetic construct
  source 1..21: mol_type = other RNA
  misc_feature 21: note = n is a,g,c or u
gtggcagccccttggtgttan

SEQ ID NO: 208 - RNA, 21 nt, synthetic construct
  source 1..21: mol_type = other RNA
  misc_feature 21: note = n is a,g,c or u
ggcagccccttggtgttatan

SEQ ID NO: 209 - RNA, 21 nt, synthetic construct
  source 1..21: mol_type = other RNA
  misc_feature 21: note = n is a,g,c or u
gacacgatgctcagatgcagn

SEQ ID NO: 210 - RNA, 21 nt, synthetic construct
  source 1..21: mol_type = other RNA
  misc_feature 21: note = n is a,g,c or u
cacgatgctcagatgcagaan

SEQ ID NO: 211 - RNA, 21 nt, synthetic construct
  source 1..21: mol_type = other RNA
  misc_feature 21: note = n is a,g,c or u
cgatgctcagatgcagaatgn

SEQ ID NO: 212 - RNA, 21 nt, synthetic construct
  source 1..21: mol_type = other RNA
  misc_feature 21: note = n is a,g,c or u
ctcagatgcagaatggactgn

SEQ ID NO: 213 - RNA, 21 nt, synthetic construct
  source 1..21: mol_type = other RNA
  misc_feature 21: note = n is a,g,c or u
ccttcgtccctccgaatgttn

SEQ ID NO: 214 - RNA, 21 nt, synthetic construct
  source 1..21: mol_type = other RNA
  misc_feature 21: note = n is a,g,c or u
cttcgtccctccgaatgttan

SEQ ID NO: 215 - RNA, 21 nt, synthetic construct
  source 1..21: mol_type = other RNA
  misc_feature 21: note = n is a,g,c or u
cgtccctccgaatgttattcn

SEQ ID NO: 216 - RNA, 21 nt, synthetic construct
  source 1..21: mol_type = other RNA
  misc_feature 21: note = n is a,g,c or u
ctccaagcctagaggcttttn

SEQ ID NO: 217 - RNA, 21 nt, synthetic construct
  source 1..21: mol_type = other RNA
  misc_feature 21: note = n is a,g,c or u
ccaagcctagaggcttttttn

SEQ ID NO: 218 - RNA, 21 nt, synthetic construct
  source 1..21: mol_type = other RNA
  misc_feature 21: note = n is a,g,c or u
caagcctagaggctttttttn

SEQ ID NO: 219 - RNA, 21 nt, synthetic construct
  source 1..21: mol_type = other RNA
  misc_feature 21: note = n is a,g,c or u
gcctagaggctttttttgaan

SEQ ID NO: 220 - RNA, 21 nt, synthetic construct
  source 1..21: mol_type = other RNA
  misc_feature 21: note = n is a,g,c or u
cctagaggctttttttgaacn

SEQ ID NO: 221 - RNA, 21 nt, synthetic construct
  source 1..21: mol_type = other RNA
  misc_feature 21: note = n is a,g,c or u
ggctttttttgaacaagcacn

SEQ ID NO: 222 - RNA, 21 nt, synthetic construct
  source 1..21: mol_type = other RNA
  misc_feature 21: note = n is a,g,c or u
ctttttttgaacaagcactgn

SEQ ID NO: 223 - RNA, 21 nt, synthetic construct
  source 1..21: mol_type = other RNA
  misc_feature 21: note = n is a,g,c or u
caagcactgactgaggaaacn

SEQ ID NO: 224 - RNA, 21 nt, synthetic construct
  source 1..21: mol_type = other RNA
  misc_feature 21: note = n is a,g,c or u
ccggggtacaggactgctacn

SEQ ID NO: 225 - RNA, 21 nt, synthetic construct
  source 1..21: mol_type = other RNA
  misc_feature 21: note = n is a,g,c or u
ggggtacaggactgctactan

SEQ ID NO: 226 - RNA, 21 nt, synthetic construct
  source 1..21: mol_type = other RNA
  misc_feature 21: note = n is a,g,c or u
gggtacaggactgctactacn

SEQ ID NO: 227 - RNA, 21 nt, synthetic construct
  source 1..21: mol_type = other RNA
  misc_feature 21: note = n is a,g,c or u
caggactgctactaccattan

SEQ ID NO: 228 - RNA, 21 nt, synthetic construct
  source 1..21: mol_type = other RNA
  misc_feature 21: note = n is a,g,c or u
ggactgctactaccattatgn

SEQ ID NO: 229 - RNA, 21 nt, synthetic construct
  source 1..21: mol_type = other RNA
  misc_feature 21: note = n is a,g,c or u
ctgctactaccattatggacn

SEQ ID NO: 230 - RNA, 21 nt, synthetic construct
  source 1..21: mol_type = other RNA
  misc_feature 21: note = n is a,g,c or u
gctactaccattatggacagn

SEQ ID NO: 231 - RNA, 21 nt, synthetic construct
  source 1..21: mol_type = other RNA
  misc_feature 21: note = n is a,g,c or u
ctaccattatggacagagttn

SEQ ID NO: 232 - RNA, 21 nt, synthetic construct
  source 1..21: mol_type = other RNA
  misc_feature 21: note = n is a,g,c or u
cacaatgcctggtgacagaan

SEQ ID NO: 233 - RNA, 21 nt, synthetic construct
  source 1..21: mol_type = other RNA
  misc_feature 21: note = n is a,g,c or u
caatgcctggtgacagaatcn

SEQ ID NO: 234 - RNA, 21 nt, synthetic construct
  source 1..21: mol_type = other RNA
  misc_feature 21: note = n is a,g,c or u
cctggtgacagaatcaagtgn

SEQ ID NO: 235 - RNA, 21 nt, synthetic construct
  source 1..21: mol_type = other RNA
  misc_feature 21: note = n is a,g,c or u
caagtgtccttgcaactctcn

SEQ ID NO: 236 - RNA, 21 nt, synthetic construct
  source 1..21: mol_type = other RNA
  misc_feature 21: note = n is a,g,c or u
cacggtggtcccagatccaan

SEQ ID NO: 237 - RNA, 21 nt, synthetic construct
  source 1..21: mol_type = other RNA
  misc_feature 21: note = n is a,g,c or u
cagaggcttcttctgaagaan

SEQ ID NO: 238 - RNA, 21 nt, synthetic construct
  source 1..21: mol_type = other RNA
  misc_feature 21: note = n is a,g,c or u
ggcttcttctgaagaagcacn

SEQ ID NO: 239 - RNA, 21 nt, synthetic construct
  source 1..21: mol_type = other RNA
  misc_feature 21: note = n is a,g,c or u
cccggggtccaggattgctan

SEQ ID NO: 240 - RNA, 21 nt, synthetic construct
  source 1..21: mol_type = other RNA
  misc_feature 21: note = n is a,g,c or u
ccggggtccaggattgctacn

SEQ ID NO: 241 - RNA, 21 nt, synthetic construct
  source 1..21: mol_type = other RNA
  misc_feature 21: note = n is a,g,c or u
ctggcatcagaggacaacagn

SEQ ID NO: 242 - RNA, 21 nt, synthetic construct
  source 1..21: mol_type = other RNA
  misc_feature 21: note = n is a,g,c or u
ggcatcagaggacaacagaan

SEQ ID NO: 243 - RNA, 21 nt, synthetic construct
  source 1..21: mol_type = other RNA
  misc_feature 21: note = n is a,g,c or u
gcatcagaggacaacagaatn

SEQ ID NO: 244 - RNA, 21 nt, synthetic construct
  source 1..21: mol_type = other RNA
  misc_feature 21: note = n is a,g,c or u
catcagaggacaacagaatan

SEQ ID NO: 245 - RNA, 21 nt, synthetic construct
  source 1..21: mol_type = other RNA
  misc_feature 21: note = n is a,g,c or u
cagaggacaacagaatattan

SEQ ID NO: 246 - RNA, 21 nt, synthetic construct
  source 1..21: mol_type = other RNA
  misc_feature 21: note = n is a,g,c or u
gaggacaacagaatattatcn

SEQ ID NO: 247 - RNA, 21 nt, synthetic construct
  source 1..21: mol_type = other RNA
  misc_feature 21: note = n is a,g,c or u
gacaacagaatattatccaan

SEQ ID NO: 248 - RNA, 21 nt, synthetic construct
  source 1..21: mol_type = other RNA
  misc_feature 21: note = n is a,g,c or u
caacagaatattatccaaatn

SEQ ID NO: 249 - RNA, 21 nt, synthetic construct
  source 1..21: mol_type = other RNA
  misc_feature 21: note = n is a,g,c or u
gatgctgagattagtccttgn

SEQ ID NO: 250 - RNA, 21 nt, synthetic construct
  source 1..21: mol_type = other RNA
  misc_feature 21: note = n is a,g,c or u
gagattagtccttggtgttan

SEQ ID NO: 251 - RNA, 21 nt, synthetic construct
  source 1..21: mol_type = other RNA
  misc_feature 21: note = n is a,g,c or u
gattagtccttggtgttatan

SEQ ID NO: 252 - RNA, 21 nt, synthetic construct
  source 1..21: mol_type = other RNA
  misc_feature 21: note = n is a,g,c or u
gtccttggtgttataccatgn

SEQ ID NO: 253 - RNA, 21 nt, synthetic construct
  source 1..21: mol_type = other RNA
  misc_feature 21: note = n is a,g,c or u
gcgacgtccacggctgtttcn

SEQ ID NO: 254 - RNA, 21 nt, synthetic construct
  source 1..21: mol_type = other RNA
  misc_feature 21: note = n is a,g,c or u
gacgtccacggctgtttctgn

SEQ ID NO: 255 - RNA, 21 nt, synthetic construct
  source 1..21: mol_type = other RNA
  misc_feature 21: note = n is a,g,c or u
cgtccacggctgtttctgaan

SEQ ID NO: 256 - RNA, 21 nt, synthetic construct
  source 1..21: mol_type = other RNA
  misc_feature 21: note = n is a,g,c or u
gtccacggctgtttctgaacn

SEQ ID NO: 257 - RNA, 21 nt, synthetic construct
  source 1..21: mol_type = other RNA
  misc_feature 21: note = n is a,g,c or u
ccacggctgtttctgaacaan

SEQ ID NO: 258 - RNA, 21 nt, synthetic construct
  source 1..21: mol_type = other RNA
  misc_feature 21: note = n is a,g,c or u
cacggctgtttctgaacaagn

SEQ ID NO: 259 - RNA, 21 nt, synthetic construct
  source 1..21: mol_type = other RNA
  misc_feature 21: note = n is a,g,c or u
ggctgtttctgaacaagcacn

SEQ ID NO: 260 - RNA, 21 nt, synthetic construct
  source 1..21: mol_type = other RNA
  misc_feature 21: note = n is a,g,c or u
ccacagtccaggactgctacn

SEQ ID NO: 261 - RNA, 21 nt, synthetic construct
  source 1..21: mol_type = other RNA
  misc_feature 21: note = n is a,g,c or u
ctggcatcagagaaccacagn

SEQ ID NO: 262 - RNA, 21 nt, synthetic construct
  source 1..21: mol_type = other RNA
  misc_feature 21: note = n is a,g,c or u
catcagagaaccacagaatan

SEQ ID NO: 263 - RNA, 21 nt, synthetic construct
  source 1..21: mol_type = other RNA
  misc_feature 21: note = n is a,g,c or u
cagagaaccacagaatactan

SEQ ID NO: 264 - RNA, 21 nt, synthetic construct
  source 1..21: mol_type = other RNA
  misc_feature 21: note = n is a,g,c or u
cgcaatgtccagtgatggaan

SEQ ID NO: 265 - RNA, 21 nt, synthetic construct
  source 1..21: mol_type = other RNA
  misc_feature 21: note = n is a,g,c or u
gcaatgtccagtgatggaatn

SEQ ID NO: 266 - RNA, 21 nt, synthetic construct
  source 1..21: mol_type = other RNA
  misc_feature 21: note = n is a,g,c or u
caatgtccagtgatggaatcn

SEQ ID NO: 267 - RNA, 21 nt, synthetic construct
  source 1..21: mol_type = other RNA
  misc_feature 21: note = n is a,g,c or u
cagtgatggaatcaactctcn

SEQ ID NO: 268 - RNA, 21 nt, synthetic construct
  source 1..21: mol_type = other RNA
  misc_feature 21: note = n is a,g,c or u
gaatcaactctcctcacaacn

SEQ ID NO: 269 - RNA, 21 nt, synthetic construct
  source 1..21: mol_type = other RNA
  misc_feature 21: note = n is a,g,c or u
ccaagcacagagcttccttcn

SEQ ID NO: 270 - RNA, 21 nt, synthetic construct
  source 1..21: mol_type = other RNA
  misc_feature 21: note = n is a,g,c or u
gcacagagcttccttctgaan

SEQ ID NO: 271 - RNA, 21 nt, synthetic construct
  source 1..21: mol_type = other RNA
  misc_feature 21: note = n is a,g,c or u
cacagagcttccttctgaagn

SEQ ID NO: 272 - RNA, 21 nt, synthetic construct
  source 1..21: mol_type = other RNA
  misc_feature 21: note = n is a,g,c or u
cagagcttccttctgaagaan

SEQ ID NO: 273 - RNA, 21 nt, synthetic construct
  source 1..21: mol_type = other RNA
  misc_feature 21: note = n is a,g,c or u
gcttccttctgaagaagcacn

SEQ ID NO: 274 - RNA, 21 nt, synthetic construct
  source 1..21: mol_type = other RNA
  misc_feature 21: note = n is a,g,c or u
gaagaagcaccaactgaaaan

SEQ ID NO: 275 - RNA, 21 nt, synthetic construct
  source 1..21: mol_type = other RNA
  misc_feature 21: note = n is a,g,c or u
gaagcaccaactgaaaacagn

SEQ ID NO: 276 - RNA, 21 nt, synthetic construct
  source 1..21: mol_type = other RNA
  misc_feature 21: note = n is a,g,c or u
gcaccaactgaaaacagcacn

SEQ ID NO: 277 - RNA, 21 nt, synthetic construct
  source 1..21: mol_type = other RNA
  misc_feature 21: note = n is a,g,c or u
ctggggtccaggactgctacn

SEQ ID NO: 278 - RNA, 21 nt, synthetic construct
  source 1..21: mol_type = other RNA
  misc_feature 21: note = n is a,g,c or u
ggactgctaccgaggtgatgn

SEQ ID NO: 279 - RNA, 21 nt, synthetic construct
  source 1..21: mol_type = other RNA
  misc_feature 21: note = n is a,g,c or u
ctgctaccgaggtgatggacn

SEQ ID NO: 280 - RNA, 21 nt, synthetic construct
  source 1..21: mol_type = other RNA
  misc_feature 21: note = n is a,g,c or u
gctaccgaggtgatggacagn

SEQ ID NO: 281 - RNA, 21 nt, synthetic construct
  source 1..21: mol_type = other RNA
  misc_feature 21: note = n is a,g,c or u
ccgaggtgatggacagagttn

SEQ ID NO: 282 - RNA, 21 nt, synthetic construct
  source 1..21: mol_type = other RNA
  misc_feature 21: note = n is a,g,c or u
cgaggtgatggacagagttan

SEQ ID NO: 283 - RNA, 21 nt, synthetic construct
  source 1..21: mol_type = other RNA
  misc_feature 21: note = n is a,g,c or u
gaggtgatggacagagttatn

SEQ ID NO: 284 - RNA, 21 nt, synthetic construct
  source 1..21: mol_type = other RNA
  misc_feature 21: note = n is a,g,c or u
gcacactctccaccactatcn

SEQ ID NO: 285 - RNA, 21 nt, synthetic construct
  source 1..21: mol_type = other RNA
  misc_feature 21: note = n is a,g,c or u
ggcatcggaggatcccattan

SEQ ID NO: 286 - RNA, 21 nt, synthetic construct
  source 1..21: mol_type = other RNA
  misc_feature 21: note = n is a,g,c or u
gcatcggaggatcccattatn

SEQ ID NO: 287 - RNA, 21 nt, synthetic construct
  source 1..21: mol_type = other RNA
  misc_feature 21: note = n is a,g,c or u
catcggaggatcccattatan

SEQ ID NO: 288 - RNA, 21 nt, synthetic construct
  source 1..21: mol_type = other RNA
  misc_feature 21: note = n is a,g,c or u
cggaggatcccattatactan

SEQ ID NO: 289 - RNA, 21 nt, synthetic construct
  source 1..21: mol_type = other RNA
  misc_feature 21: note = n is a,g,c or u
ggaggatcccattatactatn

SEQ ID NO: 290 - RNA, 21 nt, synthetic construct
  source 1..21: mol_type = other RNA
  misc_feature 21: note = n is a,g,c or u
gaggatcccattatactatcn

SEQ ID NO: 291 - RNA, 21 nt, synthetic construct
  source 1..21: mol_type = other RNA
  misc_feature 21: note = n is a,g,c or u
gatcccattatactatccaan

SEQ ID NO: 292 - RNA, 21 nt, synthetic construct
  source 1..21: mol_type = other RNA
  misc_feature 21: note = n is a,g,c or u
cccattatactatccaaatgn

SEQ ID NO: 293 - RNA, 21 nt, synthetic construct
  source 1..21: mol_type = other RNA
  misc_feature 21: note = n is a,g,c or u
gaatcgagtgtcctcacaacn

SEQ ID NO: 294 - RNA, 21 nt, synthetic construct
  source 1..21: mol_type = other RNA
  misc_feature 21: note = n is a,g,c or u
ggccccggttccaagcacagn

SEQ ID NO: 295 - RNA, 21 nt, synthetic construct
  source 1..21: mol_type = other RNA
  misc_feature 21: note = n is a,g,c or u
caagcaccacctgagaaaagn

SEQ ID NO: 296 - RNA, 21 nt, synthetic construct
  source 1..21: mol_type = other RNA
  misc_feature 21: note = n is a,g,c or u
cggagttatcgaggcatatcn

SEQ ID NO: 297 - RNA, 21 nt, synthetic construct
  source 1..21: mol_type = other RNA
  misc_feature 21: note = n is a,g,c or u
gctggcctgaccgagaactan

SEQ ID NO: 298 - RNA, 21 nt, synthetic construct
  source 1..21: mol_type = other RNA
  misc_feature 21: note = n is a,g,c or u
ctggcctgaccgagaactacn

SEQ ID NO: 299 - RNA, 21 nt, synthetic construct
  source 1..21: mol_type = other RNA
  misc_feature 21: note = n is a,g,c or u
ggcctgaccgagaactactgn

SEQ ID NO: 300 - RNA, 21 nt, synthetic construct
  source 1..21: mol_type = other RNA
  misc_feature 21: note = n is a,g,c or u
ctgaccgagaactactgcagn

SEQ ID NO: 301 - RNA, 21 nt, synthetic construct
  source 1..21: mol_type = other RNA
  misc_feature 21: note = n is a,g,c or u
cgagaactactgcaggaatcn

SEQ ID NO: 302 - RNA, 21 nt, synthetic construct
  source 1..21: mol_type = other RNA
  misc_feature 21: note = n is a,g,c or u
cagaatcaggtgtcctagagn

SEQ ID NO: 303 - RNA, 21 nt, synthetic construct
  source 1..21: mol_type = other RNA
  misc_feature 21: note = n is a,g,c or u
gaatcaggtgtcctagagacn

SEQ ID NO: 304 - RNA, 21 nt, synthetic construct
  source 1..21: mol_type = other RNA
  misc_feature 21: note = n is a,g,c or u
gcctagggcctccttctgaan

SEQ ID NO: 305 - RNA, 21 nt, synthetic construct
  source 1..21: mol_type = other RNA
  misc_feature 21: note = n is a,g,c or u
cctagggcctccttctgaacn

SEQ ID NO: 306 - RNA, 21 nt, synthetic construct
  source 1..21: mol_type = other RNA
  misc_feature 21: note = n is a,g,c or u
ggcctccttctgaacaagacn

SEQ ID NO: 307 - RNA, 21 nt, synthetic construct
  source 1..21: mol_type = other RNA
  misc_feature 21: note = n is a,g,c or u
cctccttctgaacaagactgn

SEQ ID NO: 308 - RNA, 21 nt, synthetic construct
  source 1..21: mol_type = other RNA
  misc_feature 21: note = n is a,g,c or u
ccttctgaacaagactgtatn

SEQ ID NO: 309 - RNA, 21 nt, synthetic construct
  source 1..21: mol_type = other RNA
  misc_feature 21: note = n is a,g,c or u
cttctgaacaagactgtatgn

SEQ ID NO: 310 - RNA, 21 nt, synthetic construct
  source 1..21: mol_type = other RNA
  misc_feature 21: note = n is a,g,c or u
ctgaacaagactgtatgtttn

SEQ ID NO: 311 - RNA, 21 nt, synthetic construct
  source 1..21: mol_type = other RNA
  misc_feature 21: note = n is a,g,c or u
cgttcattccagggacaaatn

SEQ ID NO: 312 - RNA, 21 nt, synthetic construct
  source 1..21: mol_type = other RNA
  misc_feature 21: note = n is a,g,c or u
gttcattccagggacaaatan

SEQ ID NO: 313 - RNA, 21 nt, synthetic construct
  source 1..21: mol_type = other RNA
  misc_feature 21: note = n is a,g,c or u
cattccagggacaaataaatn

SEQ ID NO: 314 - RNA, 21 nt, synthetic construct
  source 1..21: mol_type = other RNA
  misc_feature 21: note = n is a,g,c or u
gtaaccctgatggtgacatcn

SEQ ID NO: 315 - RNA, 21 nt, synthetic construct
  source 1..21: mol_type = other RNA
  misc_feature 21: note = n is a,g,c or u
ccctgatggtgacatcaatgn

SEQ ID NO: 316 - RNA, 21 nt, synthetic construct
  source 1..21: mol_type = other RNA
  misc_feature 21: note = n is a,g,c or u
ctggtgctacacaatgaatcn

SEQ ID NO: 317 - RNA, 21 nt, synthetic construct
  source 1..21: mol_type = other RNA
  misc_feature 21: note = n is a,g,c or u
gtgctacacaatgaatccaan

SEQ ID NO: 318 - RNA, 21 nt, synthetic construct
  source 1..21: mol_type = other RNA
  misc_feature 21: note = n is a,g,c or u
ctacacaatgaatccaagaan

SEQ ID NO: 319 - RNA, 21 nt, synthetic construct
  source 1..21: mol_type = other RNA
  misc_feature 21: note = n is a,g,c or u
cacaatgaatccaagaaaacn

SEQ ID NO: 320 - RNA, 21 nt, synthetic construct
  source 1..21: mol_type = other RNA
  misc_feature 21: note = n is a,g,c or u
gaatccaagaaaactttttgn

SEQ ID NO: 321 - RNA, 21 nt, synthetic construct
  source 1..21: mol_type = other RNA
  misc_feature 21: note = n is a,g,c or u
ccaagaaaactttttgactan

SEQ ID NO: 322 - RNA, 21 nt, synthetic construct
  source 1..21: mol_type = other RNA
  misc_feature 21: note = n is a,g,c or u
caagaaaactttttgactacn

SEQ ID NO: 323 - RNA, 21 nt, synthetic construct
  source 1..21: mol_type = other RNA
  misc_feature 21: note = n is a,g,c or u
ctttttgactactgtgatatn

SEQ ID NO: 324 - RNA, 21 nt, synthetic construct
  source 1..21: mol_type = other RNA
  misc_feature 21: note = n is a,g,c or u
ctgtgatatccctctctgtgn

SEQ ID NO: 325 - RNA, 21 nt, synthetic construct
  source 1..21: mol_type = other RNA
  misc_feature 21: note = n is a,g,c or u
ctgtgcatcctcttcatttgn

SEQ ID NO: 326 - RNA, 21 nt, synthetic construct
  source 1..21: mol_type = other RNA
  misc_feature 21: note = n is a,g,c or u
gaaatgtcctggaagcattgn

SEQ ID NO: 327 - RNA, 21 nt, synthetic construct
  source 1..21: mol_type = other RNA
  misc_feature 21: note = n is a,g,c or u
ctgctgctcactgcttgaagn

SEQ ID NO: 328 - RNA, 21 nt, synthetic construct
  source 1..21: mol_type = other RNA
  misc_feature 21: note = n is a,g,c or u
gctgctcactgcttgaagaan

SEQ ID NO: 329 - RNA, 21 nt, synthetic construct
  source 1..21: mol_type = other RNA
  misc_feature 21: note = n is a,g,c or u
ctgctcactgcttgaagaagn

SEQ ID NO: 330 - RNA, 21 nt, synthetic construct
  source 1..21: mol_type = other RNA
  misc_feature 21: note = n is a,g,c or u
gctcactgcttgaagaagtcn

SEQ ID NO: 331 - RNA, 21 nt, synthetic construct
  source 1..21: mol_type = other RNA
  misc_feature 21: note = n is a,g,c or u
cactgcttgaagaagtcctcn

SEQ ID NO: 332 - RNA, 21 nt, synthetic construct
  source 1..21: mol_type = other RNA
  misc_feature 21: note = n is a,g,c or u
gaacctcgaatctcatgttcn

SEQ ID NO: 333 - RNA, 21 nt, synthetic construct
  source 1..21: mol_type = other RNA
  misc_feature 21: note = n is a,g,c or u
cgaatctcatgttcaggaaan

SEQ ID NO: 334 - RNA, 21 nt, synthetic construct
  source 1..21: mol_type = other RNA
  misc_feature 21: note = n is a,g,c or u
gaatctcatgttcaggaaatn

SEQ ID NO: 335 - RNA, 21 nt, synthetic construct
  source 1..21: mol_type = other RNA
  misc_feature 21: note = n is a,g,c or u
ctcatgttcaggaaatagaan

SEQ ID NO: 336 - RNA, 21 nt, synthetic construct
  source 1..21: mol_type = other RNA
  misc_feature 21: note = n is a,g,c or u
cttggagcccacacaagcagn

SEQ ID NO: 337 - RNA, 21 nt, synthetic construct
  source 1..21: mol_type = other RNA
  misc_feature 21: note = n is a,g,c or u
ggagcccacacaagcagatan

SEQ ID NO: 338 - RNA, 21 nt, synthetic construct
  source 1..21: mol_type = other RNA
  misc_feature 21: note = n is a,g,c or u
gagcccacacaagcagatatn

SEQ ID NO: 339 - RNA, 21 nt, synthetic construct
  source 1..21: mol_type = other RNA
  misc_feature 21: note = n is a,g,c or u
gcccacacaagcagatattgn

SEQ ID NO: 340 - RNA, 21 nt, synthetic construct
  source 1..21: mol_type = other RNA
  misc_feature 21: note = n is a,g,c or u
cacaagcagatattgccttgn

SEQ ID NO: 341 - RNA, 21 nt, synthetic construct
  source 1..21: mol_type = other RNA
  misc_feature 21: note = n is a,g,c or u
gcagatattgccttgctaaan

SEQ ID NO: 342 - RNA, 21 nt, synthetic construct
  source 1..21: mol_type = other RNA
  misc_feature 21: note = n is a,g,c or u
gtctgccatccccagactacn

SEQ ID NO: 343 - RNA, 21 nt, synthetic construct
  source 1..21: mol_type = other RNA
  misc_feature 21: note = n is a,g,c or u
ctgccatccccagactacatn

SEQ ID NO: 344 - RNA, 21 nt, synthetic construct
  source 1..21: mol_type = other RNA
  misc_feature 21: note = n is a,g,c or u
catccccagactacatggtcn

SEQ ID NO: 345 - RNA, 21 nt, synthetic construct
  source 1..21: mol_type = other RNA
  misc_feature 21: note = n is a,g,c or u
ggtcaccgccaggactgaatn

SEQ ID NO: 346 - RNA, 21 nt, synthetic construct
  source 1..21: mol_type = other RNA
  misc_feature 21: note = n is a,g,c or u
gtcaccgccaggactgaatgn

SEQ ID NO: 347 - RNA, 21 nt, synthetic construct
  source 1..21: mol_type = other RNA
  misc_feature 21: note = n is a,g,c or u
caccgccaggactgaatgttn

SEQ ID NO: 348 - RNA, 21 nt, synthetic construct
  source 1..21: mol_type = other RNA
  misc_feature 21: note = n is a,g,c or u
ccgccaggactgaatgttacn

SEQ ID NO: 349 - RNA, 21 nt, synthetic construct
  source 1..21: mol_type = other RNA
  misc_feature 21: note = n is a,g,c or u
gccaggactgaatgttacatn

SEQ ID NO: 350 - RNA, 21 nt, synthetic construct
  source 1..21: mol_type = other RNA
  misc_feature 21: note = n is a,g,c or u
ccaggactgaatgttacatcn

SEQ ID NO: 351 - RNA, 21 nt, synthetic construct
  source 1..21: mol_type = other RNA
  misc_feature 21: note = n is a,g,c or u
gaagcccagctccttgttatn

SEQ ID NO: 352 - RNA, 21 nt, synthetic construct
  source 1..21: mol_type = other RNA
  misc_feature 21: note = n is a,g,c or u
cccagctccttgttattgagn

SEQ ID NO: 353 - RNA, 21 nt, synthetic construct
  source 1..21: mol_type = other RNA
  misc_feature 21: note = n is a,g,c or u
cagctccttgttattgagaan

SEQ ID NO: 354 - RNA, 21 nt, synthetic construct
  source 1..21: mol_type = other RNA
  misc_feature 21: note = n is a,g,c or u
gctccttgttattgagaatgn

SEQ ID NO: 355 - RNA, 21 nt, synthetic construct
  source 1..21: mol_type = other RNA
  misc_feature 21: note = n is a,g,c or u
ccttgttattgagaatgaagn

SEQ ID NO: 356 - RNA, 21 nt, synthetic construct
  source 1..21: mol_type = other RNA
  misc_feature 21: note = n is a,g,c or u
gttattgagaatgaagtgtgn

SEQ ID NO: 357 - RNA, 21 nt, synthetic construct
  source 1..21: mol_type = other RNA
  misc_feature 21: note = n is a,g,c or u
gaagtgtgcaatcactataan

SEQ ID NO: 358 - RNA, 21 nt, synthetic construct
  source 1..21: mol_type = other RNA
  misc_feature 21: note = n is a,g,c or u
gtgtgcaatcactataagtan

SEQ ID NO: 359 - RNA, 21 nt, synthetic construct
  source 1..21: mol_type = other RNA
  misc_feature 21: note = n is a,g,c or u
gtgcaatcactataagtatan

SEQ ID NO: 360 - RNA, 21 nt, synthetic construct
  source 1..21: mol_type = other RNA
  misc_feature 21: note = n is a,g,c or u
gcaatcactataagtatattn

SEQ ID NO: 361 - RNA, 21 nt, synthetic construct
  source 1..21: mol_type = other RNA
  misc_feature 21: note = n is a,g,c or u
caatcactataagtatatttn

SEQ ID NO: 362 - RNA, 21 nt, synthetic construct
  source 1..21: mol_type = other RNA
  misc_feature 21: note = n is a,g,c or u
ctataagtatatttgtgctgn

SEQ ID NO: 363 - RNA, 21 nt, synthetic construct
  source 1..21: mol_type = other RNA
  misc_feature 21: note = n is a,g,c or u
gtatatttgtgctgagcattn

SEQ ID NO: 364 - RNA, 21 nt, synthetic construct
  source 1..21: mol_type = other RNA
  misc_feature 21: note = n is a,g,c or u
gagacagagtgaagcatcaan

SEQ ID NO: 365 - RNA, 21 nt, synthetic construct
  source 1..21: mol_type = other RNA
  misc_feature 21: note = n is a,g,c or u
cagagtgaagcatcaacctan

SEQ ID NO: 366 - RNA, 21 nt, synthetic construct
  source 1..21: mol_type = other RNA
  misc_feature 21: note = n is a,g,c or u
gtgaagcatcaacctacttan

SEQ ID NO: 367 - RNA, 21 nt, synthetic construct
  source 1..21: mol_type = other RNA
  misc_feature 21: note = n is a,g,c or u
caacctacttagaagctgaan

SEQ ID NO: 368 - RNA, 21 nt, synthetic construct
  source 1..21: mol_type = other RNA
  misc_feature 21: note = n is a,g,c or u
gaagctgaaacgtgggtaagn

SEQ ID NO: 369 - RNA, 21 nt, synthetic construct
  source 1..21: mol_type = other RNA
  misc_feature 21: note = n is a,g,c or u
gctgaaacgtgggtaaggatn

SEQ ID NO: 370 - RNA, 21 nt, synthetic construct
  source 1..21: mol_type = other RNA
  misc_feature 21: note = n is a,g,c or u
ctgaaacgtgggtaaggattn

SEQ ID NO: 371 - RNA, 21 nt, synthetic construct
  source 1..21: mol_type = other RNA
  misc_feature 21: note = n is a,g,c or u
gaaacgtgggtaaggatttan

SEQ ID NO: 372 - RNA, 21 nt, synthetic construct
  source 1..21: mol_type = other RNA
  misc_feature 21: note = n is a,g,c or u
ggaaataatagacagcaatcn

SEQ ID NO: 373 - RNA, 21 nt, synthetic construct
  source 1..21: mol_type = other RNA
  misc_feature 21: note = n is a,g,c or u
gacagcaatcaaacgaagacn

SEQ ID NO: 374 - RNA, 21 nt, synthetic construct
  source 1..21: mol_type = other RNA
  misc_feature 21: note = n is a,g,c or u
ctatgccaaaccttggcattn

SEQ ID NO: 375 - RNA, 21 nt, synthetic construct
  source 1..21: mol_type = other RNA
  misc_feature 21: note = n is a,g,c or u
gccaaaccttggcatttttgn

SEQ ID NO: 376 - RNA, 21 nt, synthetic construct
  source 1..21: mol_type = other RNA
  misc_feature 21: note = n is a,g,c or u
ccttggcatttttggtatttn

SEQ ID NO: 377 - RNA, 21 nt, synthetic construct
  source 1..21: mol_type = other RNA
  misc_feature 21: note = n is a,g,c or u
cttggcatttttggtattttn

SEQ ID NO: 378 - RNA, 21 nt, synthetic construct
  source 1..21: mol_type = other RNA
  misc_feature 21: note = n is a,g,c or u
gcatttttggtatttttgtgn

SEQ ID NO: 379 - RNA, 21 nt, synthetic construct
  source 1..21: mol_type = other RNA
  misc_feature 21: note = n is a,g,c or u
gtatttttgtgtataagcttn

SEQ ID NO: 380 - RNA, 21 nt, synthetic construct
  source 1..21: mol_type = other RNA
  misc_feature 21: note = n is a,g,c or u
gtgtataagcttttaaggtcn

SEQ ID NO: 381 - RNA, 21 nt, synthetic construct
  source 1..21: mol_type = other RNA
  misc_feature 21: note = n is a,g,c or u
gtataagcttttaaggtctgn

SEQ ID NO: 382 - RNA, 21 nt, synthetic construct
  source 1..21: mol_type = other RNA
  misc_feature 21: note = n is a,g,c or u
gcttttaaggtctgactgacn

SEQ ID NO: 383 - RNA, 21 nt, synthetic construct
  source 1..21: mol_type = other RNA
  misc_feature 21: note = n is a,g,c or u
ggtctgactgacaaattctgn

SEQ ID NO: 384 - RNA, 21 nt, synthetic construct
  source 1..21: mol_type = other RNA
  misc_feature 21: note = n is a,g,c or u
ctgactgacaaattctgtatn

SEQ ID NO: 385 - RNA, 21 nt, synthetic construct
  source 1..21: mol_type = other RNA
  misc_feature 21: note = n is a,g,c or u
gactgacaaattctgtattan

SEQ ID NO: 386 - RNA, 21 nt, synthetic construct
  source 1..21: mol_type = other RNA
  misc_feature 21: note = n is a,g,c or u
ctgacaaattctgtattaagn

SEQ ID NO: 387 - RNA, 21 nt, synthetic construct
  source 1..21: mol_type = other RNA
  misc_feature 21: note = n is a,g,c or u
gtattaaggtgtcatagctan

SEQ ID NO: 388 - RNA, 21 nt, synthetic construct
  source 1..21: mol_type = other RNA
  misc_feature 21: note = n is a,g,c or u
ctctgcacttattttgatttn

SEQ ID NO: 389 - RNA, 19 nt, synthetic construct
  source 1..19: mol_type = other RNA
gacatttgttaaaaataaa

SEQ ID NO: 390 - RNA, 19 nt, synthetic construct
  source 1..19: mol_type = other RNA
gaatgatgagaaataatta

SEQ ID NO: 391 - RNA, 19 nt, synthetic construct
  source 1..19: mol_type = other RNA
gggcaggtctggaaaaaaa

SEQ ID NO: 392 - RNA, 19 nt, synthetic construct
  source 1..19: mol_type = other RNA
ggttcttctacttctttta

SEQ ID NO: 393 - RNA, 19 nt, synthetic construct
  source 1..19: mol_type = other RNA
ggacaaatacattttacaa

SEQ ID NO: 394 - RNA, 19 nt, synthetic construct
  source 1..19: mol_type = other RNA
ggaggatcccattatacta

SEQ ID NO: 395 - RNA, 19 nt, synthetic construct
  source 1..19: mol_type = other RNA
ccttgttattgagaatgaa

SEQ ID NO: 396 - RNA, 21 nt, synthetic construct
  source 1..21: mol_type = other RNA
tggtaatggacagagttattt

SEQ ID NO: 397 - RNA, 21 nt, synthetic construct
  source 1..21: mol_type = other RNA
acagagttatcgaggctcatt

SEQ ID NO: 398 - RNA, 21 nt, synthetic construct
  source 1..21: mol_type = other RNA
gtaatggacagagttatcgat

SEQ ID NO: 399 - RNA, 19 nt, synthetic construct
  source 1..19: mol_type = other RNA
gccccttggtgttatacaa

SEQ ID NO: 400 - RNA, 19 nt, synthetic construct
  source 1..19: mol_type = other RNA
gctccttattgttatacga

SEQ ID NO: 401 - RNA, 21 nt, synthetic construct
  source 1..21: mol_type = other RNA
catggtaatggacagagttat

SEQ ID NO: 402 - RNA, 21 nt, synthetic construct
  source 1..21: mol_type = other RNA
ggacagagttatcgaggctca

SEQ ID NO: 403 - RNA, 21 nt, synthetic construct
  source 1..21: mol_type = other RNA
agagttatcgaggctcattat

SEQ ID NO: 404 - RNA, 19 nt, synthetic construct
  source 1..19: mol_type = other RNA
gaaggacaaatacatttta

SEQ ID NO: 405 - RNA, 19 nt, synthetic construct
  source 1..19: mol_type = other RNA
cgttcattccagggacaaa

SEQ ID NO: 406 - RNA, 19 nt, synthetic construct
  source 1..19: mol_type = other RNA
cgtgtttcaaggtttgtta

SEQ ID NO: 407 - RNA, 21 nt, synthetic construct
  source 1..21: mol_type = other RNA
tttatttttaacaaatgtcat

SEQ ID NO: 408 - RNA, 21 nt, synthetic construct
  source 1..21: mol_type = other RNA
taattatttctcatcattccc

SEQ ID NO: 409 - RNA, 21 nt, synthetic construct
  source 1..21: mol_type = other RNA
tttttttccagacctgcccat

SEQ ID NO: 410 - RNA, 21 nt, synthetic construct
  source 1..21: mol_type = other RNA
taaaagaagtagaagaaccac

SEQ ID NO: 411 - RNA, 21 nt, synthetic construct
  source 1..21: mol_type = other RNA
ttgtaaaatgtatttgtcctt

SEQ ID NO: 412 - RNA, 21 nt, synthetic construct
  source 1..21: mol_type = other RNA
tagtataatgggatcctccga

SEQ ID NO: 413 - RNA, 21 nt, synthetic construct
  source 1..21: mol_type = other RNA
ttcattctcaataacaaggag

SEQ ID NO: 414 - RNA, 21 nt, synthetic construct
  source 1..21: mol_type = other RNA
ataactctgtccattaccatt

SEQ ID NO: 415 - RNA, 21 nt, synthetic construct
  source 1..21: mol_type = other RNA
tgagcctcgataactctgttt

SEQ ID NO: 416 - RNA, 21 nt, synthetic construct
  source 1..21: mol_type = other RNA
cgataactctgtccattacca

SEQ ID NO: 417 - RNA, 21 nt, synthetic construct
  source 1..21: mol_type = other RNA
ttgtataacaccaaggggctg

SEQ ID NO: 418 - RNA, 21 nt, synthetic construct
  source 1..21: mol_type = other RNA
tcgtataacaataaggagctg

SEQ ID NO: 419 - RNA, 21 nt, synthetic construct
  source 1..21: mol_type = other RNA
aactctgtccattaccatgtt

SEQ ID NO: 420 - RNA, 21 nt, synthetic construct
  source 1..21: mol_type = other RNA
agcctcgataactctgtcctt

SEQ ID NO: 421 - RNA, 21 nt, synthetic construct
  source 1..21: mol_type = other RNA
aatgagcctcgataactctgt

SEQ ID NO: 422 - RNA, 21 nt, synthetic construct
  source 1..21: mol_type = other RNA
taaaatgtatttgtccttctc

SEQ ID NO: 423 - RNA, 21 nt, synthetic construct
  source 1..21: mol_type = other RNA
tttgtccctggaatgaacgtg

SEQ ID NO: 424 - RNA, 21 nt, synthetic construct
  source 1..21: mol_type = other RNA
taacaaaccttgaaacacgag

SEQ ID NO: 425 - RNA, 19 nt, synthetic construct
  source 1..19: mol_type = other RNA
  misc_feature 1..19: note = 2' -OH of the nucleotides at positions 1, 2, 4, 8, 11-15, 17-19 from the 5' end of the sense strand is replaced by methoxy group
gacatttgttaaaaataaa

SEQ ID NO: 426 - RNA, 19 nt, synthetic construct
  source 1..19: mol_type = other RNA
  misc_feature 1..19: note = 2' -OH of the nucleotides at positions 1-3, 5-6, 8-13, 15-16, 19 from the 5' end of the sense strand is replaced by methoxy group
gaatgatgagaaataatta

SEQ ID NO: 427 - RNA, 19 nt, synthetic construct
  source 1..19: mol_type = other RNA
  misc_feature 1..19: note = 2' -OH of the nucleotides at positions 1-3, 5-7, 11-19 from the 5' end of the sense strand is replaced by methoxy group
gggcaggtctggaaaaaaa

SEQ ID NO: 428 - RNA, 19 nt, synthetic construct
  source 1..19: mol_type = other RNA
  misc_feature 1..19: note = 2' -OH of the nucleotides at positions 1-2, 10, 19 from the 5' end of the sense strand is replaced by methoxy group
ggttcttctacttctttta

SEQ ID NO: 429 - RNA, 19 nt, synthetic construct
  source 1..19: mol_type = other RNA
  misc_feature 1..19: note = 2' -OH of the nucleotides at positions 1-3, 5-7, 9, 11, 16, 18-19 from the 5' end of the sense strand is replaced by methoxy group
ggacaaatacattttacaa

SEQ ID NO: 430 - RNA, 19 nt, synthetic construct
  source 1..19: mol_type = other RNA
  misc_feature 1..19: note = 2' -OH of the nucleotides at positions 1-6, 11, 14, 16, 19 from the 5' end of the sense strand is replaced by methoxy group
ggaggatcccattatacta

SEQ ID NO: 431 - RNA, 19 nt, synthetic construct
  source 1..19: mol_type = other RNA
  misc_feature 1..19: note = 2' -OH of the nucleotides at positions 5, 8, 11-15, 17-19 from the 5' end of the sense strand is replaced by methoxy group
ccttgttattgagaatgaa

SEQ ID NO: 432 - RNA, 19 nt, synthetic construct
  source 1..19: mol_type = other RNA
  misc_feature 1..19: note = 2' -OH of the nucleotides at positions 1-6, 8-10, 12, 14, 19 from the 5' end of the sense strand is replaced by methoxy group
gaaggacaaatacatttta

SEQ ID NO: 433 - RNA, 19 nt, synthetic construct
  source 1..19: mol_type = other RNA
  misc_feature 1..19: note = 2' -OH of the nucleotides at positions 1, 8-9, 11, 14 , 16, 18-19 from the 5' end of the sense strand is replaced by methoxy group
gccccttggtgttatacaa

SEQ ID NO: 434 - RNA, 19 nt, synthetic construct
  source 1..19: mol_type = other RNA
  misc_feature 1..19: note = 2' -OH of the nucleotides at positions 2, 6, 11-15, 17-19 from the 5' end of the sense strand is replaced by methoxy group
cgttcattccagggacaaa

SEQ ID NO: 435 - RNA, 19 nt, synthetic construct
  source 1..19: mol_type = other RNA
  misc_feature 1..19: note = 2' -OH of the nucleotides at positions 1, 8, 11, 14, 16, 18-19 from the 5' end of the sense strand is replaced by methoxy group
gctccttattgttatacga

SEQ ID NO: 436 - RNA, 19 nt, synthetic construct
  source 1..19: mol_type = other RNA
  misc_feature 1..19: note = 2' -OH of the nucleotides at positions 2, 4, 9-12, 16, 19 from the 5' end of the sense strand is replaced by methoxy group
cgtgtttcaaggtttgtta

SEQ ID NO: 437 - RNA, 21 nt, synthetic construct
  source 1..21: mol_type = other RNA
  misc_feature 1..21: note = 2' -OH of the nucleotides at positions 1, 2, 4-8, 10-11, 13-15 ,17-18, 20-21 from the 5' end of the antisense strand is replaced by methoxy group
tttatttttaacaaatgtcat

SEQ ID NO: 438 - RNA, 21 nt, synthetic construct
  source 1..21: mol_type = other RNA
  misc_feature 1..21: note = 2' -OH of the nucleotides at positions 2-4, 6-11, 13-14, 16-21 from the 5' end of the antisense strand is replaced by methoxy group
taattatttctcatcattccc

SEQ ID NO: 439 - RNA, 21 nt, synthetic construct
  source 1..21: mol_type = other RNA
  misc_feature 1..21: note = 2' -OH of the nucleotides at positions 1-8, 10-14, 16-18, 20-21 from the 5' end of the antisense strand is replaced by methoxy group
tttttttccagacctgcccat

SEQ ID NO: 440 - RNA, 21 nt, synthetic construct
  source 1..21: mol_type = other RNA
  misc_feature 1..21: note = 2' -OH of the nucleotides at positions 2-9, 11-18, 20-21 from the 5' end of the antisense strand is replaced by methoxy group
taaaagaagtagaagaaccac

SEQ ID NO: 441 - RNA, 21 nt, synthetic construct
  source 1..21: mol_type = other RNA
  misc_feature 1..21: note = 2' -OH of the nucleotides at positions 1, 3, 5-8, 10, 12-14, 16-21 from the 5' end of the antisense strand is replaced by methoxy group
ttgtaaaatgtatttgtcctt

SEQ ID NO: 442 - RNA, 21 nt, synthetic construct
  source 1..21: mol_type = other RNA
  misc_feature 1..21: note = 2' -OH of the nucleotides at positions 2-3, 5, 7-8, 10-21 from the 5' end of the antisense strand is replaced by methoxy group
tagtataatgggatcctccga

SEQ ID NO: 443 - RNA, 21 nt, synthetic construct
  source 1..21: mol_type = other RNA
  misc_feature 1..21: note = 2' -OH of the nucleotides at positions 1-2, 4-8, 10-11, 13-21 from the 5' end of the antisense strand is replaced by methoxy group
ttcattctcaataacaaggag

SEQ ID NO: 444 - RNA, 21 nt, synthetic construct
  source 1..21: mol_type = other RNA
  misc_feature 1..21: note = 2' -OH of the nucleotides at positions 2-5, 7, 9-11, 13-21 from the 5' end of the antisense strand is replaced by methoxy group
taaaatgtatttgtccttctc

SEQ ID NO: 445 - RNA, 21 nt, synthetic construct
  source 1..21: mol_type = other RNA
  misc_feature 1..21: note = 2' -OH of the nucleotides at positions 1, 3, 5, 7-8, 10-11, 13-19, 21 from the 5' end of the antisense strand is replaced by methoxy group
ttgtataacaccaaggggctg

SEQ ID NO: 446 - RNA, 21 nt, synthetic construct
  source 1..21: mol_type = other RNA
  misc_feature 1..21: note = 2' -OH of the nucleotides at positions 1-2, 4-8, 10-19, 21 from the 5' end of the antisense strand is replaced by methoxy group
tttgtccctggaatgaacgtg

SEQ ID NO: 447 - RNA, 21 nt, synthetic construct
  source 1..21: mol_type = other RNA
  misc_feature 1..21: note = 2' -OH of the nucleotides at positions 1-2, 4-8, 10-19, 21 from the 5' end of the antisense strand is replaced by methoxy group
tcgtataacaataaggagctg

SEQ ID NO: 448 - RNA, 21 nt, synthetic construct
  source 1..21: mol_type = other RNA
  misc_feature 1..21: note = 2' -OH of the nucleotides at positions 2-3, 5-10, 12-15, 17-21 from the 5' end of the antisense strand is replaced by methoxy group
taacaaaccttgaaacacgag

SEQ ID NO: 449 - RNA, 21 nt, synthetic construct
  source 1..21: mol_type = other RNA
  misc_feature 1..21: note = 2' -OH of the nucleotides at positions 5, 7, 8, 9, 12, 14 from the 5' end of the sense strand is replaced by fluorine, 2' -OH of the remaining nucleotides in the sense strand is replaced by methoxy group, and there are two consecutive phosphorothioate linkages between 3 adjacent nucleotides at the 5' and 3' ends of the sense strand
tggtaatggacagagttattt

SEQ ID NO: 450 - RNA, 21 nt, synthetic construct
  source 1..21: mol_type = other RNA
  misc_feature 1..21: note = 2' -OH of the nucleotides at positions 5, 7, 8, 9, 11 from the 5' end of the sense strand is replaced by fluorine, 2' -OH of the remaining nucleotides in the sense strand is replaced by methoxy group, the nucleotides at positions 1, 2 from the 3' end of the sense strand is thymidine, and there are two consecutive phosphorothioate linkages between 3 adjacent nucleotides at the 5' and 3' ends of the sense strand
acagagttatcgaggctcatt

SEQ ID NO: 451 - RNA, 21 nt, synthetic construct
  source 1..21: mol_type = other RNA
  misc_feature 1..21: note = 2' -OH of the nucleotides at positions 3, 5, 7, 8, 9, 11, 13, 15 from the 5' end of the sense strand is replaced by fluorine, 2' -OH of the remaining nucleotides in the sense strand is replaced by methoxy group, and there are two consecutive phosphorothioate linkages between 3 adjacent nucleotides at the 5' and 3' ends of the sense strand
tggtaatggacagagttattt

SEQ ID NO: 452 - RNA, 21 nt, synthetic construct
  source 1..21: mol_type = other RNA
  misc_feature 1..21: note = 2' -OH of the nucleotides at positions 3, 5, 7, 8, 9, 13, 16 from the 5' end of the sense strand is replaced by fluorine, 2' -OH of the remaining nucleotides in the sense strand is replaced by methoxy group, the nucleotides at positions 1, 2 from the 3' end of the sense strand is thymidine, and there are two consecutive phosphorothioate linkages between 3 adjacent nucleotides at the 5' and 3' ends of the sense strand
acagagttatcgaggctcatt

SEQ ID NO: 453 - RNA, 21 nt, synthetic construct
  source 1..21: mol_type = other RNA
  misc_feature 1..21: note = 2' -OH of the nucleotides at positions 5, 7, 8, 9, 11, 17 from the 5' end of the sense strand is replaced by fluorine, 2' -OH of the remaining nucleotides in the sense strand is replaced by methoxy group, and there are two consecutive phosphorothioate linkages between 3 adjacent nucleotides at the 5' and 3' ends of the sense strand
tggtaatggacagagttattt

SEQ ID NO: 454 - RNA, 21 nt, synthetic construct
  source 1..21: mol_type = other RNA
  misc_feature 1..21: note = 2' -OH of the nucleotides at positions 5, 7, 8, 9, 16 from the 5' end of the sense strand is replaced by fluorine, 2' -OH of the remaining nucleotides in the sense strand is replaced by methoxy group, the nucleotides at positions 1, 2 from the 3' end of the sense strand is thymidine, and there are two consecutive phosphorothioate linkages between 3 adjacent nucleotides at the 5' and 3' ends of the sense strand
acagagttatcgaggctcatt

SEQ ID NO: 455 - RNA, 21 nt, synthetic construct
  source 1..21: mol_type = other RNA
  misc_feature 1..21: note = 2' -OH of the nucleotides at positions5, 7, 8, 9, 15 from the 5' end of the sense strand is replaced by fluorine, 2' -OH of the remaining nucleotides in the sense strand is replaced by methoxy group, and there are two consecutive phosphorothioate linkages between 3 adjacent nucleotides at the 5' and 3' ends of the sense strand
tggtaatggacagagttattt

SEQ ID NO: 456 - RNA, 21 nt, synthetic construct
  source 1..21: mol_type = other RNA
  misc_feature 1..21: note = 2' -OH of the nucleotides at positions 5, 7, 8, 9 from the 5' end of the sense strand is replaced by fluorine, 2' -OH of the remaining nucleotides in the sense strand is replaced by methoxy group, and there are two consecutive phosphorothioate linkages between 3 adjacent nucleotides at the 5' and 3' ends of the sense strand
tggtaatggacagagttattt

SEQ ID NO: 457 - RNA, 21 nt, synthetic construct
  source 1..21: mol_type = other RNA
  misc_feature 1..21: note = 2' -OH of the nucleotides at positions 5, 7, 8, 9 from the 5' end of the sense strand is replaced by fluorine, 2' -OH of the remaining nucleotides in the sense strand is replaced by methoxy group, the nucleotides at positions 1, 2 from the 3' end of the sense strand is thymidine, and there are two consecutive phosphorothioate linkages between 3 adjacent nucleotides at the 5' and 3' ends of the sense strand
acagagttatcgaggctcatt

SEQ ID NO: 458 - RNA, 21 nt, synthetic construct
  source 1..21: mol_type = other RNA
  misc_feature 1..21: note = 2' -OH of the nucleotides at positions 3, 5, 7, 8, 9, 11, 13 from the 5' end of the sense strand is replaced by fluorine, 2' -OH of the remaining nucleotides in the sense strand is replaced by methoxy group, and there are two consecutive phosphorothioate linkages between 3 adjacent nucleotides at the 5' and 3' ends of the sense strand
gtaatggacagagttatcgat

SEQ ID NO: 459 - RNA, 21 nt, synthetic construct
  source 1..21: mol_type = other RNA
  misc_feature 1..21: note = 2' -OH of the nucleotides at positions 7, 8, 9, 14 from the 5' end of the sense strand is replaced by fluorine, 2' -OH of the remaining nucleotides in the sense strand is replaced by methoxy group, and there are two consecutive phosphorothioate linkages between 3 adjacent nucleotides at the 5' and 3' ends of the sense strand
gtaatggacagagttatcgat

SEQ ID NO: 460 - RNA, 21 nt, synthetic construct
  source 1..21: mol_type = other RNA
  misc_feature 1..21: note = 2' -OH of the nucleotides at positions 5, 7, 8, 9 from the 5' end of the sense strand is replaced by fluorine, 2' -OH of the remaining nucleotides in the sense strand is replaced by methoxy group, and there are two consecutive phosphorothioate linkages between 3 adjacent nucleotides at the 5' and 3' ends of the sense strand
gtaatggacagagttatcgat

SEQ ID NO: 461 - RNA, 19 nt, synthetic construct
  source 1..19: mol_type = other RNA
  misc_feature 1..19: note = 2' -OH of the nucleotides at positions 5, 7, 8, 9 from the 5' end of the sense strand is replaced by fluorine, 2' -OH of the remaining nucleotides in the sense strand is replaced by methoxy group, and there are two consecutive phosphorothioate linkages between 3 adjacent nucleotides at the 5' and 3' ends of the sense strand
gccccttggtgttatacaa

SEQ ID NO: 462 - RNA, 19 nt, synthetic construct
  source 1..19: mol_type = other RNA
  misc_feature 1..19: note = 2' -OH of the nucleotides at positions 5, 7, 9, 15 from the 5' end of the sense strand is replaced by fluorine, 2' -OH of the remaining nucleotides in the sense strand is replaced by methoxy group, and there are two consecutive phosphorothioate linkages between 3 adjacent nucleotides at the 5' and 3' ends of the sense strand
gccccttggtgttatacaa

SEQ ID NO: 463 - RNA, 19 nt, synthetic construct
  source 1..19: mol_type = other RNA
  misc_feature 1..19: note = 2' -OH of the nucleotides at positions 3, 5, 7, 8, 9, 11, 13, 15 from the 5' end of the sense strand is replaced by fluorine, 2' -OH of the remaining nucleotides in the sense strand is replaced by methoxy group, and there are two consecutive phosphorothioate linkages between 3 adjacent nucleotides at the 5' and 3' ends of the sense strand
gccccttggtgttatacaa

SEQ ID NO: 464 - RNA, 19 nt, synthetic construct
  source 1..19: mol_type = other RNA
  misc_feature 1..19: note = 2' -OH of the nucleotides at positions 5, 7, 8, 9 from the 5' end of the sense strand is replaced by fluorine, 2' -OH of the remaining nucleotides in the sense strand is replaced by methoxy group, and there are two consecutive phosphorothioate linkages between 3 adjacent nucleotides at the 5' and 3' ends of the sense strand
gctccttattgttatacga

SEQ ID NO: 465 - RNA, 19 nt, synthetic construct
  source 1..19: mol_type = other RNA
  misc_feature 1..19: note = 2' -OH of the nucleotides at positions 3, 5, 7, 8, 9, 11, 13, 15 from the 5' end of the sense strand is replaced by fluorine, 2' -OH of the remaining nucleotides in the sense strand is replaced by methoxy group, and there are two consecutive phosphorothioate linkages between 3 adjacent nucleotides at the 5' and 3' ends of the sense strand
gctccttattgttatacga

SEQ ID NO: 466 - RNA, 21 nt, synthetic construct
  source 1..21: mol_type = other RNA
  misc_feature 1..21: note = 2' -OH of the nucleotides at positions 5, 7, 8, 9, 15 from the 5' end of the sense strand is replaced by fluorine, 2' -OH of the remaining nucleotides in the sense strand is replaced by methoxy group, and there are two consecutive phosphorothioate linkages between 3 adjacent nucleotides at the 5' and 3' ends of the sense strand
gtaatggacagagttatcgat

SEQ ID NO: 467 - RNA, 21 nt, synthetic construct
  source 1..21: mol_type = other RNA
  misc_feature 1..21: note = 2' -OH of the nucleotides at positions 7, 8, 9 from the 5' end of the sense strand is replaced by fluorine, 2' -OH of the remaining nucleotides in the sense strand is replaced by methoxy group, and there are two consecutive phosphorothioate linkages between 3 adjacent nucleotides at the 5' and 3' ends of the sense strand
gtaatggacagagttatcgat

SEQ ID NO: 468 - RNA, 21 nt, synthetic construct
  source 1..21: mol_type = other RNA
  misc_feature 1..21: note = 2' -OH of the nucleotides at positions 5, 7, 8, 9, 19 from the 5' end of the sense strand is replaced by fluorine, 2' -OH of the remaining nucleotides in the sense strand is replaced by methoxy group, and there are two consecutive phosphorothioate linkages between 3 adjacent nucleotides at the 5' and 3' ends of the sense strand
gtaatggacagagttatcgat

SEQ ID NO: 469 - RNA, 21 nt, synthetic construct
  source 1..21: mol_type = other RNA
  misc_feature 1..21: note = 2' -OH of the nucleotides at positions 3, 5, 7, 8, 9 from the 5' end of the sense strand is replaced by fluorine, 2' -OH of the remaining nucleotides in the sense strand is replaced by methoxy group, and there are two consecutive phosphorothioate linkages between 3 adjacent nucleotides at the 5' and 3' ends of the sense strand
gtaatggacagagttatcgat

SEQ ID NO: 470 - RNA, 21 nt, synthetic construct
  source 1..21: mol_type = other RNA
  misc_feature 1..21: note = 2' -OH of the nucleotides at positions 2, 5, 7, 8, 9 from the 5' end of the sense strand is replaced by fluorine, 2' -OH of the remaining nucleotides in the sense strand is replaced by methoxy group, and there are two consecutive phosphorothioate linkages between 3 adjacent nucleotides at the 5' and 3' ends of the sense strand
gtaatggacagagttatcgat

SEQ ID NO: 471 - RNA, 21 nt, synthetic construct
  source 1..21: mol_type = other RNA
  misc_feature 1..21: note = 2' -OH of the nucleotides at positions 2, 5, 7, 9 from the 5' end of the sense strand is replaced by fluorine, 2' -OH of the remaining nucleotides in the sense strand is replaced by methoxy group, and there are two consecutive phosphorothioate linkages between 3 adjacent nucleotides at the 5' and 3' ends of the sense strand
gtaatggacagagttatcgat

SEQ ID NO: 472 - RNA, 21 nt, synthetic construct
  source 1..21: mol_type = other RNA
  misc_feature 1..21: note = 2' -OH of the nucleotides at positions 5, 7, 8, 9, 10 from the 5' end of the sense strand is replaced by fluorine, 2' -OH of the remaining nucleotides in the sense strand is replaced by methoxy group, and there are two consecutive phosphorothioate linkages between 3 adjacent nucleotides at the 5' and 3' ends of the sense strand
gtaatggacagagttatcgat

SEQ ID NO: 473 - RNA, 21 nt, synthetic construct
  source 1..21: mol_type = other RNA
  misc_feature 1..21: note = 2' -OH of the nucleotides at positions 7, 9, 10, 11 from the 5' end of the sense strand is replaced by fluorine, 2' -OH of the remaining nucleotides in the sense strand is replaced by methoxy group, and there are two consecutive phosphorothioate linkages between 3 adjacent nucleotides at the 5' and 3' ends of the sense strand
gtaatggacagagttatcgat

SEQ ID NO: 474 - RNA, 21 nt, synthetic construct
  source 1..21: mol_type = other RNA
  misc_feature 1..21: note = 2' -OH of the nucleotides at positions 7, 10, 11, 12 from the 5' end of the sense strand is replaced by fluorine, 2' -OH of the remaining nucleotides in the sense strand is replaced by methoxy group, and there are two consecutive phosphorothioate linkages between 3 adjacent nucleotides at the 5' and 3' ends of the sense strand
gtaatggacagagttatcgat

SEQ ID NO: 475 - RNA, 21 nt, synthetic construct
  source 1..21: mol_type = other RNA
  misc_feature 1..21: note = 2' -OH of the nucleotides at positions 5, 7, 9, 10 from the 5' end of the sense strand is replaced by fluorine, 2' -OH of the remaining nucleotides in the sense strand is replaced by methoxy group, and there are two consecutive phosphorothioate linkages between 3 adjacent nucleotides at the 5' and 3' ends of the sense strand
gtaatggacagagttatcgat

SEQ ID NO: 476 - RNA, 21 nt, synthetic construct
  source 1..21: mol_type = other RNA
  misc_feature 1..21: note = 2' -OH of the nucleotides at positions 7, 8, 9, 15 from the 5' end of the sense strand is replaced by fluorine, 2' -OH of the remaining nucleotides in the sense strand is replaced by methoxy group, and there are two consecutive phosphorothioate linkages between 3 adjacent nucleotides at the 5' and 3' ends of the sense strand
gtaatggacagagttatcgat

SEQ ID NO: 477 - RNA, 21 nt, synthetic construct
  source 1..21: mol_type = other RNA
  misc_feature 1..21: note = 2' -OH of the nucleotides at positions 1, 3, 5, 7, 8, 9, 12, 14, 16 from the 5' end of the sense strand is replaced by fluorine, 2' -OH of the remaining nucleotides in the sense strand is replaced by methoxy group, and there are two consecutive phosphorothioate linkages between 3 adjacent nucleotides at the 5' and 3' ends of the sense strand
gtaatggacagagttatcgat

SEQ ID NO: 478 - RNA, 21 nt, synthetic construct
  source 1..21: mol_type = other RNA
  misc_feature 1..21: note = 2' -OH of the nucleotides at positions 5, 7, 8, 9, 14 from the 5' end of the sense strand is replaced by fluorine, 2' -OH of the remaining nucleotides in the sense strand is replaced by methoxy group, and there are two consecutive phosphorothioate linkages between 3 adjacent nucleotides at the 5' and 3' ends of the sense strand
gtaatggacagagttatcgat

SEQ ID NO: 479 - RNA, 21 nt, synthetic construct
  source 1..21: mol_type = other RNA
  misc_feature 1..21: note = 2' -OH of the nucleotides at positions 8, 9 from the 5' end of the sense strand is replaced by fluorine, 2' -OH of the remaining nucleotides in the sense strand is replaced by methoxy group, and there are two consecutive phosphorothioate linkages between 3 adjacent nucleotides at the 5' and 3' ends of the sense strand
gtaatggacagagttatcgat

SEQ ID NO: 480 - RNA, 19 nt, synthetic construct
  source 1..19: mol_type = other RNA
  misc_feature 1..19: note = 2' -OH of the nucleotides at positions 8, 9, 14 from the 5' end of the sense strand is replaced by fluorine, 2' -OH of the remaining nucleotides in the sense strand is replaced by methoxy group, and there are two consecutive phosphorothioate linkages between 3 adjacent nucleotides at the 5' and 3' ends of the sense strand
gctccttattgttatacga

SEQ ID NO: 481 - RNA, 19 nt, synthetic construct
  source 1..19: mol_type = other RNA
  misc_feature 1..19: note = 2' -OH of the nucleotides at positions 7, 10, 11, 12 from the 5' end of the sense strand is replaced by fluorine, 2' -OH of the remaining nucleotides in the sense strand is replaced by methoxy group, and there are two consecutive phosphorothioate linkages between 3 adjacent nucleotides at the 5' and 3' ends of the sense strand
gctccttattgttatacga

SEQ ID NO: 482 - RNA, 21 nt, synthetic construct
  source 1..21: mol_type = other RNA
  misc_feature 1..21: note = 2' -OH of the nucleotides at positions 3, 5, 7, 8, 9, 11, 13, 15 from the 5' end of the sense strand is replaced by fluorine, 2' -OH of the remaining nucleotides in the sense strand is replaced by methoxy group, the nucleotides at positions 1, 2 from the 3' end of the sense strand is thymidine, and there are two consecutive phosphorothioate linkages between 3 adjacent nucleotides at the 5' and 3' ends of the sense strand
acagagttatcgaggctcatt

SEQ ID NO: 483 - RNA, 21 nt, synthetic construct
  source 1..21: mol_type = other RNA
  misc_feature 1..21: note = 2' -OH of the nucleotides at positions 5, 7, 8, 9, 16 from the 5' end of the sense strand is replaced by fluorine, 2' -OH of the remaining nucleotides in the sense strand is replaced by methoxy group, and there are two consecutive phosphorothioate linkages between 3 adjacent nucleotides at the 5' and 3' ends of the sense strand
gtaatggacagagttatcgat

SEQ ID NO: 484 - RNA, 19 nt, synthetic construct
  source 1..19: mol_type = other RNA
  misc_feature 1..19: note = 2' -OH of the nucleotides at positions 5, 7, 8, 9, 10 from the 5' end of the sense strand is replaced by fluorine, 2' -OH of the remaining nucleotides in the sense strand is replaced by methoxy group, and there are two consecutive phosphorothioate linkages between 3 adjacent nucleotides at the 5' and 3' ends of the sense strand
gctccttattgttatacga

SEQ ID NO: 485 - RNA, 21 nt, synthetic construct
  source 1..21: mol_type = other RNA
  misc_feature 1..21: note = 2' -OH of the nucleotides at positions 2, 6, 8, 9, 10, 14-16 from the 5' end of the antisense strand is replaced by fluorine, 2' -OH of the remaining nucleotides in the antisense strand is replaced by methoxy group, and there are two consecutive phosphorothioate linkages between 3 adjacent nucleotides at the 5' and 3' ends of the antisense strand
ataactctgtccattaccatt

SEQ ID NO: 486 - RNA, 21 nt, synthetic construct
  source 1..21: mol_type = other RNA
  misc_feature 1..21: note = 2' -OH of the nucleotides at positions 2, 6, 8, 9, 10, 14, 15, 16 from the 5' end of the antisense strand is replaced by fluorine, 2' -OH of the remaining nucleotides in the antisense strand is replaced by methoxy group, and there are two consecutive phosphorothioate linkages between 3 adjacent nucleotides at the 5' and 3' ends of the antisense strand
tgagcctcgataactctgttt

SEQ ID NO: 487 - RNA, 21 nt, synthetic construct
  source 1..21: mol_type = other RNA
  misc_feature 1..21: note = 2' -OH of the nucleotides at positions 2, 4, 6, 8, 14, 16 from the 5' end of the antisense strand is replaced by fluorine, 2' -OH of the remaining nucleotides in the antisense strand is replaced by methoxy group, and there are two consecutive phosphorothioate linkages between 3 adjacent nucleotides at the 5' and 3' ends of the antisense strand
ataactctgtccattaccatt

SEQ ID NO: 488 - RNA, 21 nt, synthetic construct
  source 1..21: mol_type = other RNA
  misc_feature 1..21: note = 2' -OH of the nucleotides at positions 4, 7, 12, 14 from the 5' end of the antisense strand is replaced by fluorine, 2' -OH of the remaining nucleotides in the antisense strand is replaced by methoxy group, and there are two consecutive phosphorothioate linkages between 3 adjacent nucleotides at the 5' and 3' ends of the antisense strand
tgagcctcgataactctgttt

SEQ ID NO: 489 - RNA, 21 nt, synthetic construct
  source 1..21: mol_type = other RNA
  misc_feature 1..21: note = 2' -OH of the nucleotides at positions 4, 7, 12, 14 from the 5' end of the antisense strand is replaced by fluorine, 2' -OH of the remaining nucleotides in the antisense strand is replaced by methoxy group, and there are two consecutive phosphorothioate linkages between 3 adjacent nucleotides at the 5' and 3' ends of the antisense strand
ataactctgtccattaccatt

SEQ ID NO: 490 - RNA, 21 nt, synthetic construct
  source 1..21: mol_type = other RNA
  misc_feature 1..21: note = 2' -OH of the nucleotides at positions 5, 7, 8, 9, 16 from the 5' end of the antisense strand is replaced by fluorine, 2' -OH of the remaining nucleotides in the antisense strand is replaced by methoxy group, and there are two consecutive phosphorothioate linkages between 3 adjacent nucleotides at the 5' and 3' ends of the antisense strand
tgagcctcgataactctgttt

SEQ ID NO: 491 - RNA, 21 nt, synthetic construct
  source 1..21: mol_type = other RNA
  misc_feature 1..21: note = 2' -OH of the nucleotides at positions 5, 7, 8, 9, 15 from the 5' end of the antisense strand is replaced by fluorine, 2' -OH of the remaining nucleotides in the antisense strand is replaced by methoxy group, and there are two consecutive phosphorothioate linkages between 3 adjacent nucleotides at the 5' and 3' ends of the antisense strand
ataactctgtccattaccatt

SEQ ID NO: 492 - RNA, 21 nt, synthetic construct
  source 1..21: mol_type = other RNA
  misc_feature 1..21: note = 2' -OH of the nucleotides at positions 7, 12, 14 from the 5' end of the antisense strand is replaced by fluorine, 2' -OH of the remaining nucleotides in the antisense strand is replaced by methoxy group, and there are two consecutive phosphorothioate linkages between 3 adjacent nucleotides at the 5' and 3' ends of the antisense strand
ataactctgtccattaccatt

SEQ ID NO: 493 - RNA, 21 nt, synthetic construct
  source 1..21: mol_type = other RNA
  misc_feature 1..21: note = 2' -OH of the nucleotides at positions 7, 12, 14 from the 5' end of the antisense strand is replaced by fluorine, 2' -OH of the remaining nucleotides in the antisense strand is replaced by methoxy group, and there are two consecutive phosphorothioate linkages between 3 adjacent nucleotides at the 5' and 3' ends of the antisense strand
tgagcctcgataactctgttt

SEQ ID NO: 494 - RNA, 21 nt, synthetic construct
  source 1..21: mol_type = other RNA
  misc_feature 1..21: note = 2' -OH of the nucleotides at positions 2, 4, 6, 8, 14, 16 from the 5' end of the antisense strand is replaced by fluorine, 2' -OH of the remaining nucleotides in the antisense strand is replaced by methoxy group, and there are two consecutive phosphorothioate linkages between 3 adjacent nucleotides at the 5' and 3' ends of the antisense strand
cgataactctgtccattacca

SEQ ID NO: 495 - RNA, 21 nt, synthetic construct
  source 1..21: mol_type = other RNA
  misc_feature 1..21: note = 2' -OH of the nucleotides at positions 7, 8, 9, 14 from the 5' end of the antisense strand is replaced by fluorine, 2' -OH of the remaining nucleotides in the antisense strand is replaced by methoxy group, and there are two consecutive phosphorothioate linkages between 3 adjacent nucleotides at the 5' and 3' ends of the antisense strand
cgataactctgtccattacca

SEQ ID NO: 496 - RNA, 21 nt, synthetic construct
  source 1..21: mol_type = other RNA
  misc_feature 1..21: note = 2' -OH of the nucleotides at positions 7, 12, 14 from the 5' end of the antisense strand is replaced by fluorine, 2' -OH of the remaining nucleotides in the antisense strand is replaced by methoxy group, and there are two consecutive phosphorothioate linkages between 3 adjacent nucleotides at the 5' and 3' ends of the antisense strand
cgataactctgtccattacca

SEQ ID NO: 497 - RNA, 21 nt, synthetic construct
  source 1..21: mol_type = other RNA
  misc_feature 1..21: note = 2' -OH of the nucleotides at positions 7, 12, 14 from the 5' end of the antisense strand is replaced by fluorine, 2' -OH of the remaining nucleotides in the antisense strand is replaced by methoxy group, and there are two consecutive phosphorothioate linkages between 3 adjacent nucleotides at the 5' and 3' ends of the antisense strand
ttgtataacaccaaggggctg

SEQ ID NO: 498 - RNA, 21 nt, synthetic construct
  source 1..21: mol_type = other RNA
  misc_feature 1..21: note = 2' -OH of the nucleotides at positions 5, 7, 9, 14 from the 5' end of the antisense strand is replaced by fluorine, 2' -OH of the remaining nucleotides in the antisense strand is replaced by methoxy group, and there are two consecutive phosphorothioate linkages between 3 adjacent nucleotides at the 5' and 3' ends of the antisense strand
ttgtataacaccaaggggctg

SEQ ID NO: 499 - RNA, 21 nt, synthetic construct
  source 1..21: mol_type = other RNA
  misc_feature 1..21: note = 2' -OH of the nucleotides at positions 2, 4, 6, 8, 14, 16 from the 5' end of the antisense strand is replaced by fluorine, 2' -OH of the remaining nucleotides in the antisense strand is replaced by methoxy group, and there are two consecutive phosphorothioate linkages between 3 adjacent nucleotides at the 5' and 3' ends of the antisense strand
ttgtataacaccaaggggctg

SEQ ID NO: 500 - RNA, 21 nt, synthetic construct
  source 1..21: mol_type = other RNA
  misc_feature 1..21: note = 2' -OH of the nucleotides at positions 7, 12, 14 from the 5' end of the antisense strand is replaced by fluorine, 2' -OH of the remaining nucleotides in the antisense strand is replaced by methoxy group, and there are two consecutive phosphorothioate linkages between 3 adjacent nucleotides at the 5' and 3' ends of the antisense strand
tcgtataacaataaggagctg

SEQ ID NO: 501 - RNA, 21 nt, synthetic construct
  source 1..21: mol_type = other RNA
  misc_feature 1..21: note = 2' -OH of the nucleotides at positions 2, 4, 6, 8, 14, 16 from the 5' end of the antisense strand is replaced by fluorine, 2' -OH of the remaining nucleotides in the antisense strand is replaced by methoxy group, and there are two consecutive phosphorothioate linkages between 3 adjacent nucleotides at the 5' and 3' ends of the antisense strand
tcgtataacaataaggagctg

SEQ ID NO: 502 - RNA, 21 nt, synthetic construct
  source 1..21: mol_type = other RNA
  misc_feature 1..21: note = 2' -OH of the nucleotides at positions 5, 7, 8, 9, 15 from the 5' end of the antisense strand is replaced by fluorine, 2' -OH of the remaining nucleotides in the antisense strand is replaced by methoxy group, and there are two consecutive phosphorothioate linkages between 3 adjacent nucleotides at the 5' and 3' ends of the antisense strand
cgataactctgtccattacca

SEQ ID NO: 503 - RNA, 21 nt, synthetic construct
  source 1..21: mol_type = other RNA
  misc_feature 1..21: note = 2' -OH of the nucleotides at positions 7, 8, 9 from the 5' end of the antisense strand is replaced by fluorine, 2' -OH of the remaining nucleotides in the antisense strand is replaced by methoxy group, and there are two consecutive phosphorothioate linkages between 3 adjacent nucleotides at the 5' and 3' ends of the antisense strand
cgataactctgtccattacca

SEQ ID NO: 504 - RNA, 21 nt, synthetic construct
  source 1..21: mol_type = other RNA
  misc_feature 1..21: note = 2' -OH of the nucleotides at positions 5, 7, 8, 9 from the 5' end of the antisense strand is replaced by fluorine, 2' -OH of the remaining nucleotides in the antisense strand is replaced by methoxy group, and there are two consecutive phosphorothioate linkages between 3 adjacent nucleotides at the 5' and 3' ends of the antisense strand
cgataactctgtccattacca

SEQ ID NO: 505 - RNA, 21 nt, synthetic construct
  source 1..21: mol_type = other RNA
  misc_feature 1..21: note = 2' -OH of the nucleotides at positions 4, 5, 7, 8, 9 from the 5' end of the antisense strand is replaced by fluorine, 2' -OH of the remaining nucleotides in the antisense strand is replaced by methoxy group, and there are two consecutive phosphorothioate linkages between 3 adjacent nucleotides at the 5' and 3' ends of the antisense strand
cgataactctgtccattacca

SEQ ID NO: 506 - RNA, 21 nt, synthetic construct
  source 1..21: mol_type = other RNA
  misc_feature 1..21: note = 2' -OH of the nucleotides at positions 2, 4, 5, 7, 8, 9 from the 5' end of the antisense strand is replaced by fluorine, 2' -OH of the remaining nucleotides in the antisense strand is replaced by methoxy group, and there are two consecutive phosphorothioate linkages between 3 adjacent nucleotides at the 5' and 3' ends of the antisense strand
cgataactctgtccattacca

SEQ ID NO: 507 - RNA, 21 nt, synthetic construct
  source 1..21: mol_type = other RNA
  misc_feature 1..21: note = 2' -OH of the nucleotides at positions 2, 4, 5, 7, 9 from the 5' end of the antisense strand is replaced by fluorine, 2' -OH of the remaining nucleotides in the antisense strand is replaced by methoxy group, and there are two consecutive phosphorothioate linkages between 3 adjacent nucleotides at the 5' and 3' ends of the antisense strand
cgataactctgtccattacca

SEQ ID NO: 508 - RNA, 21 nt, synthetic construct
  source 1..21: mol_type = other RNA
  misc_feature 1..21: note = 2' -OH of the nucleotides at positions 2, 6, 8, 9, 10, 14 from the 5' end of the antisense strand is replaced by fluorine, 2' -OH of the remaining nucleotides in the antisense strand is replaced by methoxy group, and there are two consecutive phosphorothioate linkages between 3 adjacent nucleotides at the 5' and 3' ends of the antisense strand
cgataactctgtccattacca

SEQ ID NO: 509 - RNA, 21 nt, synthetic construct
  source 1..21: mol_type = other RNA
  misc_feature 1..21: note = 2' -OH of the nucleotides at positions 4, 12, 14 from the 5' end of the antisense strand is replaced by fluorine, 2' -OH of the remaining nucleotides in the antisense strand is replaced by methoxy group, and there are two consecutive phosphorothioate linkages between 3 adjacent nucleotides at the 5' and 3' ends of the antisense strand
cgataactctgtccattacca

SEQ ID NO: 510 - RNA, 21 nt, synthetic construct
  source 1..21: mol_type = other RNA
  misc_feature 1..21: note = 2' -OH of the nucleotides at positions 2, 6, 8, 10, 14, 16 from the 5' end of the antisense strand is replaced by fluorine, 2' -OH of the remaining nucleotides in the antisense strand is replaced by methoxy group, and there are two consecutive phosphorothioate linkages between 3 adjacent nucleotides at the 5' and 3' ends of the antisense strand
cgataactctgtccattacca

SEQ ID NO: 511 - RNA, 21 nt, synthetic construct
  source 1..21: mol_type = other RNA
  misc_feature 1..21: note = 2' -OH of the nucleotides at positions 2, 10, 14, 16 from the 5' end of the antisense strand is replaced by fluorine, 2' -OH of the remaining nucleotides in the antisense strand is replaced by methoxy group, and there are two consecutive phosphorothioate linkages between 3 adjacent nucleotides at the 5' and 3' ends of the antisense strand
cgataactctgtccattacca

SEQ ID NO: 512 - RNA, 21 nt, synthetic construct
  source 1..21: mol_type = other RNA
  misc_feature 1..21: note = 2' -OH of the nucleotides at positions 2, 6, 10, 14, 16 from the 5' end of the antisense strand is replaced by fluorine, 2' -OH of the remaining nucleotides in the antisense strand is replaced by methoxy group, and there are two consecutive phosphorothioate linkages between 3 adjacent nucleotides at the 5' and 3' ends of the antisense strand
cgataactctgtccattacca

SEQ ID NO: 513 - RNA, 21 nt, synthetic construct
  source 1..21: mol_type = other RNA
  misc_feature 1..21: note = 2' -OH of the nucleotides at positions 2, 4, 8, 14, 16, 18 from the 5' end of the antisense strand is replaced by fluorine, 2' -OH of the remaining nucleotides in the antisense strand is replaced by methoxy group, and there are two consecutive phosphorothioate linkages between 3 adjacent nucleotides at the 5' and 3' ends of the antisense strand
cgataactctgtccattacca

SEQ ID NO: 514 - RNA, 21 nt, synthetic construct
  source 1..21: mol_type = other RNA
  misc_feature 1..21: note = 2' -OH of the nucleotides at positions 2, 6, 8, 14, 16 from the 5' end of the antisense strand is replaced by fluorine, 2' -OH of the remaining nucleotides in the antisense strand is replaced by methoxy group, and there are two consecutive phosphorothioate linkages between 3 adjacent nucleotides at the 5' and 3' ends of the antisense strand
cgataactctgtccattacca

SEQ ID NO: 515 - RNA, 21 nt, synthetic construct
  source 1..21: mol_type = other RNA
  misc_feature 1..21: note = 2' -OH of the nucleotides at positions 2, 6, 8, 9, 10, 14, 15, 16 from the 5' end of the antisense strand is replaced by fluorine, 2' -OH of the remaining nucleotides in the antisense strand is replaced by methoxy group, and there are two consecutive phosphorothioate linkages between 3 adjacent nucleotides at the 5' and 3' ends of the antisense strand
cgataactctgtccattacca

SEQ ID NO: 516 - RNA, 21 nt, synthetic construct
  source 1..21: mol_type = other RNA
  misc_feature 1..21: note = 2' -OH of the nucleotides at positions 8, 9, 14 from the 5' end of the antisense strand is replaced by fluorine, 2' -OH of the remaining nucleotides in the antisense strand is replaced by methoxy group, and there are two consecutive phosphorothioate linkages between 3 adjacent nucleotides at the 5' and 3' ends of the antisense strand
tcgtataacaataaggagctg

SEQ ID NO: 517 - RNA, 21 nt, synthetic construct
  source 1..21: mol_type = other RNA
  misc_feature 1..21: note = 2' -OH of the nucleotides at positions 2, 14, 16 from the 5' end of the antisense strand is replaced by fluorine, 2' -OH of the remaining nucleotides in the antisense strand is replaced by methoxy group, and there are two consecutive phosphorothioate linkages between 3 adjacent nucleotides at the 5' and 3' ends of the antisense strand
tcgtataacaataaggagctg

SEQ ID NO: 518 - RNA, 21 nt, synthetic construct
  source 1..21: mol_type = other RNA
  misc_feature 1..21: note = 2' -OH of the nucleotides at positions 2, 4, 6, 8, 14, 16 from the 5' end of the antisense strand is replaced by fluorine, 2' -OH of the remaining nucleotides in the antisense strand is replaced by methoxy group, and there are two consecutive phosphorothioate linkages between 3 adjacent nucleotides at the 5' and 3' ends of the antisense strand
tgagcctcgataactctgttt

SEQ ID NO: 519 - RNA, 21 nt, synthetic construct
  source 1..21: mol_type = other RNA
  misc_feature 1..21: note = 2' -OH of the nucleotides at positions 5, 7, 8, 9, 16 from the 5' end of the antisense strand is replaced by fluorine, 2' -OH of the remaining nucleotides in the antisense strand is replaced by methoxy group, and there are two consecutive phosphorothioate linkages between 3 adjacent nucleotides at the 5' and 3' ends of the antisense strand
cgataactctgtccattacca

SEQ ID NO: 520 - RNA, 21 nt, synthetic construct
  source 1..21: mol_type = other RNA
  misc_feature 1..21: note = 2' -OH of the nucleotides at positions 2, 6, 8, 9, 10, 14 from the 5' end of the antisense strand is replaced by fluorine, 2' -OH of the remaining nucleotides in the antisense strand is replaced by methoxy group, and there are two consecutive phosphorothioate linkages between 3 adjacent nucleotides at the 5' and 3' ends of the antisense strand
tcgtataacaataaggagctg

SEQ ID NO: 521 - RNA, 21 nt, synthetic construct
  source 1..21: mol_type = other RNA
  misc_feature 1..21: note = 2' -OH of the nucleotides at positions 2, 6, 8, 9, 10, 14 from the 5' end of the antisense strand is replaced by fluorine, 2' -OH of the remaining nucleotides in the antisense strand is replaced by methoxy group, and there are two consecutive phosphorothioate linkages between 3 adjacent nucleotides at the 5' and 3' ends of the antisense strand
ttgtataacaccaaggggctg

SEQ ID NO: 522 - RNA, 21 nt, synthetic construct
  source 1..21: mol_type = other RNA
  misc_feature 1..21: note = 2' -OH of the nucleotides at positions 4, 12, 14 from the 5' end of the antisense strand is replaced by fluorine, 2' -OH of the remaining nucleotides in the antisense strand is replaced by methoxy group, and there are two consecutive phosphorothioate linkages between 3 adjacent nucleotides at the 5' and 3' ends of the antisense strand
ttgtataacaccaaggggctg

SEQ ID NO: 523 - RNA, 21 nt, synthetic construct
  source 1..21: mol_type = other RNA
  misc_feature 1..21: note = 2' -OH of the nucleotides at positions 2, 6, 8, 9, 10, 14, 15, 16 from the 5' end of the antisense strand is replaced by fluorine, 2' -OH of the remaining nucleotides in the antisense strand is replaced by methoxy group, and there are two consecutive phosphorothioate linkages between 3 adjacent nucleotides at the 5' and 3' ends of the antisense strand
ttgtataacaccaaggggctg

SEQ ID NO: 524 - RNA, 21 nt, synthetic construct
  source 1..21: mol_type = other RNA
  misc_feature 1..21: note = 2' -OH of the nucleotides at positions 4, 12, 14 from the 5' end of the antisense strand is replaced by fluorine, 2' -OH of the remaining nucleotides in the antisense strand is replaced by methoxy group, and there are two consecutive phosphorothioate linkages between 3 adjacent nucleotides at the 5' and 3' ends of the antisense strand
tcgtataacaataaggagctg

SEQ ID NO: 525 - RNA, 21 nt, synthetic construct
  source 1..21: mol_type = other RNA
  misc_feature 1..21: note = 2' -OH of the nucleotides at positions 2, 6, 8, 9, 10, 14, 15, 16 from the 5' end of the antisense strand is replaced by fluorine, 2' -OH of the remaining nucleotides in the antisense strand is replaced by methoxy group, and there are two consecutive phosphorothioate linkages between 3 adjacent nucleotides at the 5' and 3' ends of the antisense strand
tcgtataacaataaggagctg

SEQ ID NO: 526 - RNA, 21 nt, synthetic construct
  source 1..21: mol_type = other RNA
  misc_feature 1..21: note = 2' -OH of the nucleotides at positions 2, 6, 8, 10, 14, 16 from the 5' end of the antisense strand is replaced by fluorine, 2' -OH of the remaining nucleotides in the antisense strand is replaced by methoxy group, and there are two consecutive phosphorothioate linkages between 3 adjacent nucleotides at the 5' and 3' ends of the antisense strand
tcgtataacaataaggagctg

SEQ ID NO: 527 - RNA, 21 nt, synthetic construct
  source 1..21: mol_type = other RNA
  misc_feature 1..21: note = 2' -OH of the nucleotides at positions 2, 14, 16 from the 5' end of the antisense strand is replaced by fluorine, 2' -OH of the remaining nucleotides in the antisense strand is replaced by methoxy group, and there are two consecutive phosphorothioate linkages between 3 adjacent nucleotides at the 5' and 3' ends of the antisense strand
tcgtataacaataaggagctg

SEQ ID NO: 528 - RNA, 21 nt, synthetic construct
  source 1..21: mol_type = other RNA
  misc_feature 1..21: note = 2' -OH of the nucleotides at positions 2, 6, 14, 16 from the 5' end of the antisense strand is replaced by fluorine, 2' -OH of the remaining nucleotides in the antisense strand is replaced by methoxy group, and there are two consecutive phosphorothioate linkages between 3 adjacent nucleotides at the 5' and 3' ends of the antisense strand
tcgtataacaataaggagctg

SEQ ID NO: 529 - RNA, 21 nt, synthetic construct
  source 1..21: mol_type = other RNA
  misc_feature 1..21: note = 2' -OH of the nucleotides at positions 2, 4, 8, 14, 16, 18 from the 5' end of the antisense strand is replaced by fluorine, 2' -OH of the remaining nucleotides in the antisense strand is replaced by methoxy group, and there are two consecutive phosphorothioate linkages between 3 adjacent nucleotides at the 5' and 3' ends of the antisense strand
tcgtataacaataaggagctg

SEQ ID NO: 530 - RNA, 21 nt, synthetic construct
  source 1..21: mol_type = other RNA
  misc_feature 1..21: note = 2' -OH of the nucleotides at positions 2, 6, 8, 14, 16 from the 5' end of the antisense strand is replaced by fluorine, 2' -OH of the remaining nucleotides in the antisense strand is replaced by methoxy group, and there are two consecutive phosphorothioate linkages between 3 adjacent nucleotides at the 5' and 3' ends of the antisense strand
tcgtataacaataaggagctg

SEQ ID NO: 531 - RNA, 21 nt, synthetic construct
  source 1..21: mol_type = other RNA
  misc_feature 1..21: note = 2' -OH of the nucleotides at positions 2, 6, 8, 10, 14, 16 from the 5' end of the antisense strand is replaced by fluorine, 2' -OH of the remaining nucleotides in the antisense strand is replaced by methoxy group, and there are two consecutive phosphorothioate linkages between 3 adjacent nucleotides at the 5' and 3' ends of the antisense strand
ataactctgtccattaccatt

SEQ ID NO: 532 - RNA, 21 nt, synthetic construct
  source 1..21: mol_type = other RNA
  misc_feature 1..21: note = 2' -OH of the nucleotides at positions 2, 14, 16 from the 5' end of the antisense strand is replaced by fluorine, 2' -OH of the remaining nucleotides in the antisense strand is replaced by methoxy group, and there are two consecutive phosphorothioate linkages between 3 adjacent nucleotides at the 5' and 3' ends of the antisense strand
ataactctgtccattaccatt

SEQ ID NO: 533 - RNA, 21 nt, synthetic construct
  source 1..21: mol_type = other RNA
  misc_feature 1..21: note = 2' -OH of the nucleotides at positions 2, 6, 14, 16 from the 5' end of the antisense strand is replaced by fluorine, 2' -OH of the remaining nucleotides in the antisense strand is replaced by methoxy group, and there are two consecutive phosphorothioate linkages between 3 adjacent nucleotides at the 5' and 3' ends of the antisense strand
ataactctgtccattaccatt

SEQ ID NO: 534 - RNA, 21 nt, synthetic construct
  source 1..21: mol_type = other RNA
  misc_feature 1..21: note = 2' -OH of the nucleotides at positions 2, 4, 8, 14, 16, 18 from the 5' end of the antisense strand is replaced by fluorine, 2' -OH of the remaining nucleotides in the antisense strand is replaced by methoxy group, and there are two consecutive phosphorothioate linkages between 3 adjacent nucleotides at the 5' and 3' ends of the antisense strand
ataactctgtccattaccatt

SEQ ID NO: 535 - RNA, 21 nt, synthetic construct
  source 1..21: mol_type = other RNA
  misc_feature 1..21: note = 2' -OH of the nucleotides at positions 2, 6, 8, 14, 16 from the 5' end of the antisense strand is replaced by fluorine, 2' -OH of the remaining nucleotides in the antisense strand is replaced by methoxy group, and there are two consecutive phosphorothioate linkages between 3 adjacent nucleotides at the 5' and 3' ends of the antisense strand
ataactctgtccattaccatt

SEQ ID NO: 536 - RNA, 21 nt, synthetic construct
  source 1..21: mol_type = other RNA
  misc_feature 1..21: note = 2' -OH of the nucleotides at positions 2, 6, 14, 16 from the 5' end of the antisense strand is replaced by fluorine, 2' -OH of the remaining nucleotides in the antisense strand is replaced by methoxy group, and there are two consecutive phosphorothioate linkages between 3 adjacent nucleotides at the 5' and 3' ends of the antisense strand
tgagcctcgataactctgttt

SEQ ID NO: 537 - RNA, 21 nt, synthetic construct
  source 1..21: mol_type = other RNA
  misc_feature 1..21: note = 2' -OH of the nucleotides at positions 2, 4, 8, 14, 16, 18 from the 5' end of the antisense strand is replaced by fluorine, 2' -OH of the remaining nucleotides in the antisense strand is replaced by methoxy group, and there are two consecutive phosphorothioate linkages between 3 adjacent nucleotides at the 5' and 3' ends of the antisense strand
tgagcctcgataactctgttt

SEQ ID NO: 538 - RNA, 21 nt, synthetic construct
  source 1..21: mol_type = other RNA
  misc_feature 1..21: note = 2' -OH of the nucleotides at positions 2, 6, 8, 10, 14, 16 from the 5' end of the antisense strand is replaced by fluorine, 2' -OH of the remaining nucleotides in the antisense strand is replaced by methoxy group, and there are two consecutive phosphorothioate linkages between 3 adjacent nucleotides at the 5' and 3' ends of the antisense strand
tgagcctcgataactctgttt